European Patent Application EP 4 796 633 A1, published August 26, 2026. Title: 用于抑制LPA的基因表达的siRNA，含其的组合物及其用途. Applicant: 北京加科瑞康医药科技有限公司. The sequence listing filed with the application follows.

SEQUENCE LISTING (560 sequences)

SEQ ID NO: 1 - RNA, 19 nt, synthetic construct
  source 1..19: mol_type = other RNA
gtggcagctccttattgtt

SEQ ID NO: 2 - RNA, 19 nt, synthetic construct
  source 1..19: mol_type = other RNA
gcagctccttattgttata

SEQ ID NO: 3 - RNA, 19 nt, synthetic construct
  source 1..19: mol_type = other RNA
ggcagctccttattgttat

SEQ ID NO: 4 - RNA, 19 nt, synthetic construct
  source 1..19: mol_type = other RNA
gcaatgctcagacgcagaa

SEQ ID NO: 5 - RNA, 19 nt, synthetic construct
  source 1..19: mol_type = other RNA
gcttgatcaagaactactg

SEQ ID NO: 6 - RNA, 19 nt, synthetic construct
  source 1..19: mol_type = other RNA
cctagaggctccttctgaa

SEQ ID NO: 7 - RNA, 19 nt, synthetic construct
  source 1..19: mol_type = other RNA
ctccaagcctagaggcttt

SEQ ID NO: 8 - RNA, 19 nt, synthetic construct
  source 1..19: mol_type = other RNA
gatgctgagattcgccctt

SEQ ID NO: 9 - RNA, 19 nt, synthetic construct
  source 1..19: mol_type = other RNA
gcacgtactccaccactgt

SEQ ID NO: 10 - RNA, 19 nt, synthetic construct
  source 1..19: mol_type = other RNA
gaatccagatgctgagatt

SEQ ID NO: 11 - RNA, 19 nt, synthetic construct
  source 1..19: mol_type = other RNA
tggcagctccttattgtta

SEQ ID NO: 12 - RNA, 19 nt, synthetic construct
  source 1..19: mol_type = other RNA
agagttatcgaggctcatt

SEQ ID NO: 13 - RNA, 19 nt, synthetic construct
  source 1..19: mol_type = other RNA
ccttctgaacaagcaccaa

SEQ ID NO: 14 - RNA, 19 nt, synthetic construct
  source 1..19: mol_type = other RNA
actgtcacaggaagaactt

SEQ ID NO: 15 - RNA, 19 nt, synthetic construct
  source 1..19: mol_type = other RNA
ccgaacaagcaccgactga

SEQ ID NO: 16 - RNA, 19 nt, synthetic construct
  source 1..19: mol_type = other RNA
cctagaggctttttttgaa

SEQ ID NO: 17 - RNA, 19 nt, synthetic construct
  source 1..19: mol_type = other RNA
caagcaccaactgagcaaa

SEQ ID NO: 18 - RNA, 19 nt, synthetic construct
  source 1..19: mol_type = other RNA
ggacctgccaagcttggtc

SEQ ID NO: 19 - RNA, 19 nt, synthetic construct
  source 1..19: mol_type = other RNA
accattatggacagagtta

SEQ ID NO: 20 - RNA, 19 nt, synthetic construct
  source 1..19: mol_type = other RNA
gaagcaccaactgaaaaca

SEQ ID NO: 21 - RNA, 19 nt, synthetic construct
  source 1..19: mol_type = other RNA
aggactgctactaccatta

SEQ ID NO: 22 - RNA, 19 nt, synthetic construct
  source 1..19: mol_type = other RNA
ggctccttctgaacaagca

SEQ ID NO: 23 - RNA, 19 nt, synthetic construct
  source 1..19: mol_type = other RNA
aatccagatgctgagatta

SEQ ID NO: 24 - RNA, 19 nt, synthetic construct
  source 1..19: mol_type = other RNA
cactatcacaggaagaaca

SEQ ID NO: 25 - RNA, 19 nt, synthetic construct
  source 1..19: mol_type = other RNA
caagcaccgactgagcaaa

SEQ ID NO: 26 - RNA, 19 nt, synthetic construct
  source 1..19: mol_type = other RNA
ggcacgtactccaccactg

SEQ ID NO: 27 - RNA, 19 nt, synthetic construct
  source 1..19: mol_type = other RNA
gctgagattcgcccttggt

SEQ ID NO: 28 - RNA, 19 nt, synthetic construct
  source 1..19: mol_type = other RNA
ggctccttccgaacaagca

SEQ ID NO: 29 - RNA, 19 nt, synthetic construct
  source 1..19: mol_type = other RNA
agaagcaccaactgaaaac

SEQ ID NO: 30 - RNA, 19 nt, synthetic construct
  source 1..19: mol_type = other RNA
ccttctgaagaagcaccaa

SEQ ID NO: 31 - RNA, 19 nt, synthetic construct
  source 1..19: mol_type = other RNA
tgtggcagctccttattgt

SEQ ID NO: 32 - RNA, 19 nt, synthetic construct
  source 1..19: mol_type = other RNA
gagttatcgaggctcattc

SEQ ID NO: 33 - RNA, 19 nt, synthetic construct
  source 1..19: mol_type = other RNA
gaggctttttttgaacaag

SEQ ID NO: 34 - RNA, 19 nt, synthetic construct
  source 1..19: mol_type = other RNA
gcctagaggctccttctga

SEQ ID NO: 35 - RNA, 19 nt, synthetic construct
  source 1..19: mol_type = other RNA
aagaagcaccaactgaaaa

SEQ ID NO: 36 - RNA, 19 nt, synthetic construct
  source 1..19: mol_type = other RNA
acaggaagaacatgtcagt

SEQ ID NO: 37 - RNA, 19 nt, synthetic construct
  source 1..19: mol_type = other RNA
ggctgtttctgaacaagca

SEQ ID NO: 38 - RNA, 19 nt, synthetic construct
  source 1..19: mol_type = other RNA
cggtggtcccagttccaag

SEQ ID NO: 39 - RNA, 19 nt, synthetic construct
  source 1..19: mol_type = other RNA
aggacctgccaagcttggt

SEQ ID NO: 40 - RNA, 19 nt, synthetic construct
  source 1..19: mol_type = other RNA
gtcgctcctccgactgtca

SEQ ID NO: 41 - RNA, 19 nt, synthetic construct
  source 1..19: mol_type = other RNA
caggactgctactaccatt

SEQ ID NO: 42 - RNA, 19 nt, synthetic construct
  source 1..19: mol_type = other RNA
gcatcagaggacaacagaa

SEQ ID NO: 43 - RNA, 19 nt, synthetic construct
  source 1..19: mol_type = other RNA
tggcttgatcaagaactac

SEQ ID NO: 44 - RNA, 19 nt, synthetic construct
  source 1..19: mol_type = other RNA
cactggcatcagaggacaa

SEQ ID NO: 45 - RNA, 19 nt, synthetic construct
  source 1..19: mol_type = other RNA
agcctagaggctccttctg

SEQ ID NO: 46 - RNA, 19 nt, synthetic construct
  source 1..19: mol_type = other RNA
gcacagaggcttcttctga

SEQ ID NO: 47 - RNA, 19 nt, synthetic construct
  source 1..19: mol_type = other RNA
cagaatcaggtgtcctaga

SEQ ID NO: 48 - RNA, 19 nt, synthetic construct
  source 1..19: mol_type = other RNA
actatcacaggaagaacat

SEQ ID NO: 49 - RNA, 19 nt, synthetic construct
  source 1..19: mol_type = other RNA
acaggactgctactaccat

SEQ ID NO: 50 - RNA, 19 nt, synthetic construct
  source 1..19: mol_type = other RNA
ctaccattatggacagagt

SEQ ID NO: 51 - RNA, 19 nt, synthetic construct
  source 1..19: mol_type = other RNA
gcctagaggctttttttga

SEQ ID NO: 52 - RNA, 19 nt, synthetic construct
  source 1..19: mol_type = other RNA
ccgccaggactgaatgtta

SEQ ID NO: 53 - RNA, 19 nt, synthetic construct
  source 1..19: mol_type = other RNA
caagcaccaacggagcaaa

SEQ ID NO: 54 - RNA, 19 nt, synthetic construct
  source 1..19: mol_type = other RNA
cccttggtgttacaccatg

SEQ ID NO: 55 - RNA, 19 nt, synthetic construct
  source 1..19: mol_type = other RNA
ctgctactaccattatgga

SEQ ID NO: 56 - RNA, 19 nt, synthetic construct
  source 1..19: mol_type = other RNA
acaagcaccacctgagaaa

SEQ ID NO: 57 - RNA, 19 nt, synthetic construct
  source 1..19: mol_type = other RNA
caatgcctggtgacagaat

SEQ ID NO: 58 - RNA, 19 nt, synthetic construct
  source 1..19: mol_type = other RNA
aagcaccgactgagcaaag

SEQ ID NO: 59 - RNA, 19 nt, synthetic construct
  source 1..19: mol_type = other RNA
cacagaggcttcttctgaa

SEQ ID NO: 60 - RNA, 19 nt, synthetic construct
  source 1..19: mol_type = other RNA
gtgtccttgcaactctcac

SEQ ID NO: 61 - RNA, 19 nt, synthetic construct
  source 1..19: mol_type = other RNA
cagctccttattgttatac

SEQ ID NO: 62 - RNA, 19 nt, synthetic construct
  source 1..19: mol_type = other RNA
gctccttccgaacaagcac

SEQ ID NO: 63 - RNA, 19 nt, synthetic construct
  source 1..19: mol_type = other RNA
ggcatcagaggacaacaga

SEQ ID NO: 64 - RNA, 19 nt, synthetic construct
  source 1..19: mol_type = other RNA
gcaccaactgaaaacagca

SEQ ID NO: 65 - RNA, 19 nt, synthetic construct
  source 1..19: mol_type = other RNA
tgctgagattcgcccttgg

SEQ ID NO: 66 - RNA, 19 nt, synthetic construct
  source 1..19: mol_type = other RNA
ttccgaacaagcaccgact

SEQ ID NO: 67 - RNA, 19 nt, synthetic construct
  source 1..19: mol_type = other RNA
gctactaccattatggaca

SEQ ID NO: 68 - RNA, 19 nt, synthetic construct
  source 1..19: mol_type = other RNA
gcaccaactgagcaaaggc

SEQ ID NO: 69 - RNA, 19 nt, synthetic construct
  source 1..19: mol_type = other RNA
caggaagaacatgtcagtc

SEQ ID NO: 70 - RNA, 19 nt, synthetic construct
  source 1..19: mol_type = other RNA
aagcaccaacggagcaaag

SEQ ID NO: 71 - RNA, 19 nt, synthetic construct
  source 1..19: mol_type = other RNA
gacaccacaccagcatagt

SEQ ID NO: 72 - RNA, 19 nt, synthetic construct
  source 1..19: mol_type = other RNA
ctgtcacaggaagaacttg

SEQ ID NO: 73 - RNA, 19 nt, synthetic construct
  source 1..19: mol_type = other RNA
cagaggacaacagaatatt

SEQ ID NO: 74 - RNA, 19 nt, synthetic construct
  source 1..19: mol_type = other RNA
ctggcatcagaggacaaca

SEQ ID NO: 75 - RNA, 19 nt, synthetic construct
  source 1..19: mol_type = other RNA
taccattatggacagagtt

SEQ ID NO: 76 - RNA, 19 nt, synthetic construct
  source 1..19: mol_type = other RNA
tcagaggacaacagaatat

SEQ ID NO: 77 - RNA, 19 nt, synthetic construct
  source 1..19: mol_type = other RNA
catggatcccaatgtcaga

SEQ ID NO: 78 - RNA, 19 nt, synthetic construct
  source 1..19: mol_type = other RNA
ccattatggacagagttac

SEQ ID NO: 79 - RNA, 19 nt, synthetic construct
  source 1..19: mol_type = other RNA
ataccatggatcccaatgt

SEQ ID NO: 80 - RNA, 19 nt, synthetic construct
  source 1..19: mol_type = other RNA
gctccttctgaacaagcac

SEQ ID NO: 81 - RNA, 19 nt, synthetic construct
  source 1..19: mol_type = other RNA
gcaccgactgagcaaaggc

SEQ ID NO: 82 - RNA, 19 nt, synthetic construct
  source 1..19: mol_type = other RNA
tccaagcctagaggctttt

SEQ ID NO: 83 - RNA, 19 nt, synthetic construct
  source 1..19: mol_type = other RNA
tgacaccacaccagcatag

SEQ ID NO: 84 - RNA, 19 nt, synthetic construct
  source 1..19: mol_type = other RNA
cccagttccaagcacagag

SEQ ID NO: 85 - RNA, 19 nt, synthetic construct
  source 1..19: mol_type = other RNA
caccacaccagcatagtcg

SEQ ID NO: 86 - RNA, 19 nt, synthetic construct
  source 1..19: mol_type = other RNA
gtggtcccagttccaagca

SEQ ID NO: 87 - RNA, 19 nt, synthetic construct
  source 1..19: mol_type = other RNA
catcagaggacaacagaat

SEQ ID NO: 88 - RNA, 19 nt, synthetic construct
  source 1..19: mol_type = other RNA
aagcacagaggcttcttct

SEQ ID NO: 89 - RNA, 19 nt, synthetic construct
  source 1..19: mol_type = other RNA
ggtggtcccagttccaagc

SEQ ID NO: 90 - RNA, 19 nt, synthetic construct
  source 1..19: mol_type = other RNA
acaccacaccagcatagtc

SEQ ID NO: 91 - RNA, 19 nt, synthetic construct
  source 1..19: mol_type = other RNA
agcaccgactgagcaaagg

SEQ ID NO: 92 - RNA, 19 nt, synthetic construct
  source 1..19: mol_type = other RNA
ctgacacgatgtccagtga

SEQ ID NO: 93 - RNA, 19 nt, synthetic construct
  source 1..19: mol_type = other RNA
gattcgcccttggtgttac

SEQ ID NO: 94 - RNA, 19 nt, synthetic construct
  source 1..19: mol_type = other RNA
caccatggatcccagtgtc

SEQ ID NO: 95 - RNA, 19 nt, synthetic construct
  source 1..19: mol_type = other RNA
ccaagcctagaggcttttt

SEQ ID NO: 96 - RNA, 19 nt, synthetic construct
  source 1..19: mol_type = other RNA
agcacagaggcttcttctg

SEQ ID NO: 97 - RNA, 19 nt, synthetic construct
  source 1..19: mol_type = other RNA
cggctgtttctgaacaagc

SEQ ID NO: 98 - RNA, 19 nt, synthetic construct
  source 1..19: mol_type = other RNA
gtggtcccagatccaagca

SEQ ID NO: 99 - RNA, 19 nt, synthetic construct
  source 1..19: mol_type = other RNA
ccagtgacagaatcgagtg

SEQ ID NO: 100 - RNA, 19 nt, synthetic construct
  source 1..19: mol_type = other RNA
atcagaggacaacagaata

SEQ ID NO: 101 - RNA, 19 nt, synthetic construct
  source 1..19: mol_type = other RNA
aagcaccaactgagcaaag

SEQ ID NO: 102 - RNA, 19 nt, synthetic construct
  source 1..19: mol_type = other RNA
gaagaacatgtcagtcttg

SEQ ID NO: 103 - RNA, 19 nt, synthetic construct
  source 1..19: mol_type = other RNA
aagcaccaactgaaaacag

SEQ ID NO: 104 - RNA, 19 nt, synthetic construct
  source 1..19: mol_type = other RNA
aggctccttctgaacaagc

SEQ ID NO: 105 - RNA, 19 nt, synthetic construct
  source 1..19: mol_type = other RNA
agcaccaactgagcaaagg

SEQ ID NO: 106 - RNA, 19 nt, synthetic construct
  source 1..19: mol_type = other RNA
tcccacggtggtcccagtt

SEQ ID NO: 107 - RNA, 19 nt, synthetic construct
  source 1..19: mol_type = other RNA
tccgaacaagcaccgactg

SEQ ID NO: 108 - RNA, 19 nt, synthetic construct
  source 1..19: mol_type = other RNA
tccacggctgtttctgaac

SEQ ID NO: 109 - RNA, 19 nt, synthetic construct
  source 1..19: mol_type = other RNA
gaatcgagtgtcctcacaa

SEQ ID NO: 110 - RNA, 19 nt, synthetic construct
  source 1..19: mol_type = other RNA
cctgacacgatgtccagtg

SEQ ID NO: 111 - RNA, 19 nt, synthetic construct
  source 1..19: mol_type = other RNA
tcctcacaactcccacggt

SEQ ID NO: 112 - RNA, 19 nt, synthetic construct
  source 1..19: mol_type = other RNA
tggcatcagaggacaacag

SEQ ID NO: 113 - RNA, 19 nt, synthetic construct
  source 1..19: mol_type = other RNA
ggacaacagaatattatcc

SEQ ID NO: 114 - RNA, 19 nt, synthetic construct
  source 1..19: mol_type = other RNA
ggtggtcccagatccaagc

SEQ ID NO: 115 - RNA, 19 nt, synthetic construct
  source 1..19: mol_type = other RNA
aggcttcttctgaagaagc

SEQ ID NO: 116 - RNA, 19 nt, synthetic construct
  source 1..19: mol_type = other RNA
tctcacggtggtcccagat

SEQ ID NO: 117 - RNA, 19 nt, synthetic construct
  source 1..19: mol_type = other RNA
actggcatcagaggacaac

SEQ ID NO: 118 - RNA, 19 nt, synthetic construct
  source 1..19: mol_type = other RNA
ggtgttataccatggatcc

SEQ ID NO: 119 - RNA, 19 nt, synthetic construct
  source 1..19: mol_type = other RNA
acaccatggatcccagtgt

SEQ ID NO: 120 - RNA, 19 nt, synthetic construct
  source 1..19: mol_type = other RNA
ctcacggtggtcccagatc

SEQ ID NO: 121 - RNA, 19 nt, synthetic construct
  source 1..19: mol_type = other RNA
ccggttccaagcacagagg

SEQ ID NO: 122 - RNA, 19 nt, synthetic construct
  source 1..19: mol_type = other RNA
caagcacagaggcttcttc

SEQ ID NO: 123 - RNA, 19 nt, synthetic construct
  source 1..19: mol_type = other RNA
cccttggtgttataccatg

SEQ ID NO: 124 - RNA, 19 nt, synthetic construct
  source 1..19: mol_type = other RNA
ttggtgttataccatggat

SEQ ID NO: 125 - RNA, 19 nt, synthetic construct
  source 1..19: mol_type = other RNA
ggcttcttctgaagaagca

SEQ ID NO: 126 - RNA, 21 nt, synthetic construct
  source 1..21: mol_type = other RNA
acagagttatcgaggctcatt

SEQ ID NO: 127 - RNA, 21 nt, synthetic construct
  source 1..21: mol_type = other RNA
cagatgctgagattcgccctt

SEQ ID NO: 128 - RNA, 19 nt, synthetic construct
  source 1..19: mol_type = other RNA
aacaataaggagctgccac

SEQ ID NO: 129 - RNA, 19 nt, synthetic construct
  source 1..19: mol_type = other RNA
tataacaataaggagctgc

SEQ ID NO: 130 - RNA, 19 nt, synthetic construct
  source 1..19: mol_type = other RNA
ataacaataaggagctgcc

SEQ ID NO: 131 - RNA, 19 nt, synthetic construct
  source 1..19: mol_type = other RNA
ttctgcgtctgagcattgc

SEQ ID NO: 132 - RNA, 19 nt, synthetic construct
  source 1..19: mol_type = other RNA
cagtagttcttgatcaagc

SEQ ID NO: 133 - RNA, 19 nt, synthetic construct
  source 1..19: mol_type = other RNA
ttcagaaggagcctctagg

SEQ ID NO: 134 - RNA, 19 nt, synthetic construct
  source 1..19: mol_type = other RNA
aaagcctctaggcttggag

SEQ ID NO: 135 - RNA, 19 nt, synthetic construct
  source 1..19: mol_type = other RNA
aagggcgaatctcagcatc

SEQ ID NO: 136 - RNA, 19 nt, synthetic construct
  source 1..19: mol_type = other RNA
acagtggtggagtacgtgc

SEQ ID NO: 137 - RNA, 19 nt, synthetic construct
  source 1..19: mol_type = other RNA
aatctcagcatctggattc

SEQ ID NO: 138 - RNA, 19 nt, synthetic construct
  source 1..19: mol_type = other RNA
taacaataaggagctgcca

SEQ ID NO: 139 - RNA, 19 nt, synthetic construct
  source 1..19: mol_type = other RNA
aatgagcctcgataactct

SEQ ID NO: 140 - RNA, 19 nt, synthetic construct
  source 1..19: mol_type = other RNA
ttggtgcttgttcagaagg

SEQ ID NO: 141 - RNA, 19 nt, synthetic construct
  source 1..19: mol_type = other RNA
aagttcttcctgtgacagt

SEQ ID NO: 142 - RNA, 19 nt, synthetic construct
  source 1..19: mol_type = other RNA
tcagtcggtgcttgttcgg

SEQ ID NO: 143 - RNA, 19 nt, synthetic construct
  source 1..19: mol_type = other RNA
ttcaaaaaaagcctctagg

SEQ ID NO: 144 - RNA, 19 nt, synthetic construct
  source 1..19: mol_type = other RNA
tttgctcagttggtgcttg

SEQ ID NO: 145 - RNA, 19 nt, synthetic construct
  source 1..19: mol_type = other RNA
gaccaagcttggcaggtcc

SEQ ID NO: 146 - RNA, 19 nt, synthetic construct
  source 1..19: mol_type = other RNA
taactctgtccataatggt

SEQ ID NO: 147 - RNA, 19 nt, synthetic construct
  source 1..19: mol_type = other RNA
tgttttcagttggtgcttc

SEQ ID NO: 148 - RNA, 19 nt, synthetic construct
  source 1..19: mol_type = other RNA
taatggtagtagcagtcct

SEQ ID NO: 149 - RNA, 19 nt, synthetic construct
  source 1..19: mol_type = other RNA
tgcttgttcagaaggagcc

SEQ ID NO: 150 - RNA, 19 nt, synthetic construct
  source 1..19: mol_type = other RNA
taatctcagcatctggatt

SEQ ID NO: 151 - RNA, 19 nt, synthetic construct
  source 1..19: mol_type = other RNA
tgttcttcctgtgatagtg

SEQ ID NO: 152 - RNA, 19 nt, synthetic construct
  source 1..19: mol_type = other RNA
tttgctcagtcggtgcttg

SEQ ID NO: 153 - RNA, 19 nt, synthetic construct
  source 1..19: mol_type = other RNA
cagtggtggagtacgtgcc

SEQ ID NO: 154 - RNA, 19 nt, synthetic construct
  source 1..19: mol_type = other RNA
accaagggcgaatctcagc

SEQ ID NO: 155 - RNA, 19 nt, synthetic construct
  source 1..19: mol_type = other RNA
tgcttgttcggaaggagcc

SEQ ID NO: 156 - RNA, 19 nt, synthetic construct
  source 1..19: mol_type = other RNA
gttttcagttggtgcttct

SEQ ID NO: 157 - RNA, 19 nt, synthetic construct
  source 1..19: mol_type = other RNA
ttggtgcttcttcagaagg

SEQ ID NO: 158 - RNA, 19 nt, synthetic construct
  source 1..19: mol_type = other RNA
acaataaggagctgccaca

SEQ ID NO: 159 - RNA, 19 nt, synthetic construct
  source 1..19: mol_type = other RNA
gaatgagcctcgataactc

SEQ ID NO: 160 - RNA, 19 nt, synthetic construct
  source 1..19: mol_type = other RNA
cttgttcaaaaaaagcctc

SEQ ID NO: 161 - RNA, 19 nt, synthetic construct
  source 1..19: mol_type = other RNA
tcagaaggagcctctaggc

SEQ ID NO: 162 - RNA, 19 nt, synthetic construct
  source 1..19: mol_type = other RNA
ttttcagttggtgcttctt

SEQ ID NO: 163 - RNA, 19 nt, synthetic construct
  source 1..19: mol_type = other RNA
actgacatgttcttcctgt

SEQ ID NO: 164 - RNA, 19 nt, synthetic construct
  source 1..19: mol_type = other RNA
tgcttgttcagaaacagcc

SEQ ID NO: 165 - RNA, 19 nt, synthetic construct
  source 1..19: mol_type = other RNA
cttggaactgggaccaccg

SEQ ID NO: 166 - RNA, 19 nt, synthetic construct
  source 1..19: mol_type = other RNA
accaagcttggcaggtcct

SEQ ID NO: 167 - RNA, 19 nt, synthetic construct
  source 1..19: mol_type = other RNA
tgacagtcggaggagcgac

SEQ ID NO: 168 - RNA, 19 nt, synthetic construct
  source 1..19: mol_type = other RNA
aatggtagtagcagtcctg

SEQ ID NO: 169 - RNA, 19 nt, synthetic construct
  source 1..19: mol_type = other RNA
ttctgttgtcctctgatgc

SEQ ID NO: 170 - RNA, 19 nt, synthetic construct
  source 1..19: mol_type = other RNA
gtagttcttgatcaagcca

SEQ ID NO: 171 - RNA, 19 nt, synthetic construct
  source 1..19: mol_type = other RNA
ttgtcctctgatgccagtg

SEQ ID NO: 172 - RNA, 19 nt, synthetic construct
  source 1..19: mol_type = other RNA
cagaaggagcctctaggct

SEQ ID NO: 173 - RNA, 19 nt, synthetic construct
  source 1..19: mol_type = other RNA
tcagaagaagcctctgtgc

SEQ ID NO: 174 - RNA, 19 nt, synthetic construct
  source 1..19: mol_type = other RNA
tctaggacacctgattctg

SEQ ID NO: 175 - RNA, 19 nt, synthetic construct
  source 1..19: mol_type = other RNA
atgttcttcctgtgatagt

SEQ ID NO: 176 - RNA, 19 nt, synthetic construct
  source 1..19: mol_type = other RNA
atggtagtagcagtcctgt

SEQ ID NO: 177 - RNA, 19 nt, synthetic construct
  source 1..19: mol_type = other RNA
actctgtccataatggtag

SEQ ID NO: 178 - RNA, 19 nt, synthetic construct
  source 1..19: mol_type = other RNA
tcaaaaaaagcctctaggc

SEQ ID NO: 179 - RNA, 19 nt, synthetic construct
  source 1..19: mol_type = other RNA
taacattcagtcctggcgg

SEQ ID NO: 180 - RNA, 19 nt, synthetic construct
  source 1..19: mol_type = other RNA
tttgctccgttggtgcttg

SEQ ID NO: 181 - RNA, 19 nt, synthetic construct
  source 1..19: mol_type = other RNA
catggtgtaacaccaaggg

SEQ ID NO: 182 - RNA, 19 nt, synthetic construct
  source 1..19: mol_type = other RNA
tccataatggtagtagcag

SEQ ID NO: 183 - RNA, 19 nt, synthetic construct
  source 1..19: mol_type = other RNA
tttctcaggtggtgcttgt

SEQ ID NO: 184 - RNA, 19 nt, synthetic construct
  source 1..19: mol_type = other RNA
attctgtcaccaggcattg

SEQ ID NO: 185 - RNA, 19 nt, synthetic construct
  source 1..19: mol_type = other RNA
ctttgctcagtcggtgctt

SEQ ID NO: 186 - RNA, 19 nt, synthetic construct
  source 1..19: mol_type = other RNA
ttcagaagaagcctctgtg

SEQ ID NO: 187 - RNA, 19 nt, synthetic construct
  source 1..19: mol_type = other RNA
gtgagagttgcaaggacac

SEQ ID NO: 188 - RNA, 19 nt, synthetic construct
  source 1..19: mol_type = other RNA
gtataacaataaggagctg

SEQ ID NO: 189 - RNA, 19 nt, synthetic construct
  source 1..19: mol_type = other RNA
gtgcttgttcggaaggagc

SEQ ID NO: 190 - RNA, 19 nt, synthetic construct
  source 1..19: mol_type = other RNA
tctgttgtcctctgatgcc

SEQ ID NO: 191 - RNA, 19 nt, synthetic construct
  source 1..19: mol_type = other RNA
tgctgttttcagttggtgc

SEQ ID NO: 192 - RNA, 19 nt, synthetic construct
  source 1..19: mol_type = other RNA
ccaagggcgaatctcagca

SEQ ID NO: 193 - RNA, 19 nt, synthetic construct
  source 1..19: mol_type = other RNA
agtcggtgcttgttcggaa

SEQ ID NO: 194 - RNA, 19 nt, synthetic construct
  source 1..19: mol_type = other RNA
tgtccataatggtagtagc

SEQ ID NO: 195 - RNA, 19 nt, synthetic construct
  source 1..19: mol_type = other RNA
gcctttgctcagttggtgc

SEQ ID NO: 196 - RNA, 19 nt, synthetic construct
  source 1..19: mol_type = other RNA
gactgacatgttcttcctg

SEQ ID NO: 197 - RNA, 19 nt, synthetic construct
  source 1..19: mol_type = other RNA
ctttgctccgttggtgctt

SEQ ID NO: 198 - RNA, 19 nt, synthetic construct
  source 1..19: mol_type = other RNA
actatgctggtgtggtgtc

SEQ ID NO: 199 - RNA, 19 nt, synthetic construct
  source 1..19: mol_type = other RNA
caagttcttcctgtgacag

SEQ ID NO: 200 - RNA, 19 nt, synthetic construct
  source 1..19: mol_type = other RNA
aatattctgttgtcctctg

SEQ ID NO: 201 - RNA, 19 nt, synthetic construct
  source 1..19: mol_type = other RNA
tgttgtcctctgatgccag

SEQ ID NO: 202 - RNA, 19 nt, synthetic construct
  source 1..19: mol_type = other RNA
aactctgtccataatggta

SEQ ID NO: 203 - RNA, 19 nt, synthetic construct
  source 1..19: mol_type = other RNA
atattctgttgtcctctga

SEQ ID NO: 204 - RNA, 19 nt, synthetic construct
  source 1..19: mol_type = other RNA
tctgacattgggatccatg

SEQ ID NO: 205 - RNA, 19 nt, synthetic construct
  source 1..19: mol_type = other RNA
gtaactctgtccataatgg

SEQ ID NO: 206 - RNA, 19 nt, synthetic construct
  source 1..19: mol_type = other RNA
acattgggatccatggtat

SEQ ID NO: 207 - RNA, 19 nt, synthetic construct
  source 1..19: mol_type = other RNA
gtgcttgttcagaaggagc

SEQ ID NO: 208 - RNA, 19 nt, synthetic construct
  source 1..19: mol_type = other RNA
gcctttgctcagtcggtgc

SEQ ID NO: 209 - RNA, 19 nt, synthetic construct
  source 1..19: mol_type = other RNA
aaaagcctctaggcttgga

SEQ ID NO: 210 - RNA, 19 nt, synthetic construct
  source 1..19: mol_type = other RNA
ctatgctggtgtggtgtca

SEQ ID NO: 211 - RNA, 19 nt, synthetic construct
  source 1..19: mol_type = other RNA
ctctgtgcttggaactggg

SEQ ID NO: 212 - RNA, 19 nt, synthetic construct
  source 1..19: mol_type = other RNA
cgactatgctggtgtggtg

SEQ ID NO: 213 - RNA, 19 nt, synthetic construct
  source 1..19: mol_type = other RNA
tgcttggaactgggaccac

SEQ ID NO: 214 - RNA, 19 nt, synthetic construct
  source 1..19: mol_type = other RNA
attctgttgtcctctgatg

SEQ ID NO: 215 - RNA, 19 nt, synthetic construct
  source 1..19: mol_type = other RNA
agaagaagcctctgtgctt

SEQ ID NO: 216 - RNA, 19 nt, synthetic construct
  source 1..19: mol_type = other RNA
gcttggaactgggaccacc

SEQ ID NO: 217 - RNA, 19 nt, synthetic construct
  source 1..19: mol_type = other RNA
gactatgctggtgtggtgt

SEQ ID NO: 218 - RNA, 19 nt, synthetic construct
  source 1..19: mol_type = other RNA
cctttgctcagtcggtgct

SEQ ID NO: 219 - RNA, 19 nt, synthetic construct
  source 1..19: mol_type = other RNA
tcactggacatcgtgtcag

SEQ ID NO: 220 - RNA, 19 nt, synthetic construct
  source 1..19: mol_type = other RNA
gtaacaccaagggcgaatc

SEQ ID NO: 221 - RNA, 19 nt, synthetic construct
  source 1..19: mol_type = other RNA
gacactgggatccatggtg

SEQ ID NO: 222 - RNA, 19 nt, synthetic construct
  source 1..19: mol_type = other RNA
aaaaagcctctaggcttgg

SEQ ID NO: 223 - RNA, 19 nt, synthetic construct
  source 1..19: mol_type = other RNA
cagaagaagcctctgtgct

SEQ ID NO: 224 - RNA, 19 nt, synthetic construct
  source 1..19: mol_type = other RNA
gcttgttcagaaacagccg

SEQ ID NO: 225 - RNA, 19 nt, synthetic construct
  source 1..19: mol_type = other RNA
tgcttggatctgggaccac

SEQ ID NO: 226 - RNA, 19 nt, synthetic construct
  source 1..19: mol_type = other RNA
cactcgattctgtcactgg

SEQ ID NO: 227 - RNA, 19 nt, synthetic construct
  source 1..19: mol_type = other RNA
tattctgttgtcctctgat

SEQ ID NO: 228 - RNA, 19 nt, synthetic construct
  source 1..19: mol_type = other RNA
ctttgctcagttggtgctt

SEQ ID NO: 229 - RNA, 19 nt, synthetic construct
  source 1..19: mol_type = other RNA
caagactgacatgttcttc

SEQ ID NO: 230 - RNA, 19 nt, synthetic construct
  source 1..19: mol_type = other RNA
ctgttttcagttggtgctt

SEQ ID NO: 231 - RNA, 19 nt, synthetic construct
  source 1..19: mol_type = other RNA
gcttgttcagaaggagcct

SEQ ID NO: 232 - RNA, 19 nt, synthetic construct
  source 1..19: mol_type = other RNA
cctttgctcagttggtgct

SEQ ID NO: 233 - RNA, 19 nt, synthetic construct
  source 1..19: mol_type = other RNA
aactgggaccaccgtggga

SEQ ID NO: 234 - RNA, 19 nt, synthetic construct
  source 1..19: mol_type = other RNA
cagtcggtgcttgttcgga

SEQ ID NO: 235 - RNA, 19 nt, synthetic construct
  source 1..19: mol_type = other RNA
gttcagaaacagccgtgga

SEQ ID NO: 236 - RNA, 19 nt, synthetic construct
  source 1..19: mol_type = other RNA
ttgtgaggacactcgattc

SEQ ID NO: 237 - RNA, 19 nt, synthetic construct
  source 1..19: mol_type = other RNA
cactggacatcgtgtcagg

SEQ ID NO: 238 - RNA, 19 nt, synthetic construct
  source 1..19: mol_type = other RNA
accgtgggagttgtgagga

SEQ ID NO: 239 - RNA, 19 nt, synthetic construct
  source 1..19: mol_type = other RNA
ctgttgtcctctgatgcca

SEQ ID NO: 240 - RNA, 19 nt, synthetic construct
  source 1..19: mol_type = other RNA
ggataatattctgttgtcc

SEQ ID NO: 241 - RNA, 19 nt, synthetic construct
  source 1..19: mol_type = other RNA
gcttggatctgggaccacc

SEQ ID NO: 242 - RNA, 19 nt, synthetic construct
  source 1..19: mol_type = other RNA
gcttcttcagaagaagcct

SEQ ID NO: 243 - RNA, 19 nt, synthetic construct
  source 1..19: mol_type = other RNA
atctgggaccaccgtgaga

SEQ ID NO: 244 - RNA, 19 nt, synthetic construct
  source 1..19: mol_type = other RNA
gttgtcctctgatgccagt

SEQ ID NO: 245 - RNA, 19 nt, synthetic construct
  source 1..19: mol_type = other RNA
ggatccatggtataacacc

SEQ ID NO: 246 - RNA, 19 nt, synthetic construct
  source 1..19: mol_type = other RNA
acactgggatccatggtgt

SEQ ID NO: 247 - RNA, 19 nt, synthetic construct
  source 1..19: mol_type = other RNA
gatctgggaccaccgtgag

SEQ ID NO: 248 - RNA, 19 nt, synthetic construct
  source 1..19: mol_type = other RNA
cctctgtgcttggaaccgg

SEQ ID NO: 249 - RNA, 19 nt, synthetic construct
  source 1..19: mol_type = other RNA
gaagaagcctctgtgcttg

SEQ ID NO: 250 - RNA, 19 nt, synthetic construct
  source 1..19: mol_type = other RNA
catggtataacaccaaggg

SEQ ID NO: 251 - RNA, 19 nt, synthetic construct
  source 1..19: mol_type = other RNA
atccatggtataacaccaa

SEQ ID NO: 252 - RNA, 19 nt, synthetic construct
  source 1..19: mol_type = other RNA
tgcttcttcagaagaagcc

SEQ ID NO: 253 - RNA, 21 nt, synthetic construct
  source 1..21: mol_type = other RNA
aatgagcctcgataactctgt

SEQ ID NO: 254 - RNA, 21 nt, synthetic construct
  source 1..21: mol_type = other RNA
aagggcgaatctcagcatctg

SEQ ID NO: 255 - RNA, 21 nt, synthetic construct
  source 1..21: mol_type = other RNA
  misc_feature 20..21: note = T is dT
gtggcagctccttattgtttt

SEQ ID NO: 256 - RNA, 21 nt, synthetic construct
  source 1..21: mol_type = other RNA
  misc_feature 20..21: note = T is dT
gcagctccttattgttatatt

SEQ ID NO: 257 - RNA, 21 nt, synthetic construct
  source 1..21: mol_type = other RNA
  misc_feature 20..21: note = T is dT
ggcagctccttattgttattt

SEQ ID NO: 258 - RNA, 21 nt, synthetic construct
  source 1..21: mol_type = other RNA
  misc_feature 20..21: note = T is dT
gcaatgctcagacgcagaatt

SEQ ID NO: 259 - RNA, 21 nt, synthetic construct
  source 1..21: mol_type = other RNA
  misc_feature 20..21: note = T is dT
gcttgatcaagaactactgtt

SEQ ID NO: 260 - RNA, 21 nt, synthetic construct
  source 1..21: mol_type = other RNA
  misc_feature 20..21: note = T is dT
cctagaggctccttctgaatt

SEQ ID NO: 261 - RNA, 21 nt, synthetic construct
  source 1..21: mol_type = other RNA
  misc_feature 20..21: note = T is dT
ctccaagcctagaggcttttt

SEQ ID NO: 262 - RNA, 21 nt, synthetic construct
  source 1..21: mol_type = other RNA
  misc_feature 20..21: note = T is dT
gatgctgagattcgccctttt

SEQ ID NO: 263 - RNA, 21 nt, synthetic construct
  source 1..21: mol_type = other RNA
  misc_feature 20..21: note = T is dT
gcacgtactccaccactgttt

SEQ ID NO: 264 - RNA, 21 nt, synthetic construct
  source 1..21: mol_type = other RNA
  misc_feature 20..21: note = T is dT
gaatccagatgctgagatttt

SEQ ID NO: 265 - RNA, 21 nt, synthetic construct
  source 1..21: mol_type = other RNA
  misc_feature 20..21: note = T is dT
tggcagctccttattgttatt

SEQ ID NO: 266 - RNA, 21 nt, synthetic construct
  source 1..21: mol_type = other RNA
  misc_feature 20..21: note = T is dT
agagttatcgaggctcatttt

SEQ ID NO: 267 - RNA, 21 nt, synthetic construct
  source 1..21: mol_type = other RNA
  misc_feature 20..21: note = T is dT
ccttctgaacaagcaccaatt

SEQ ID NO: 268 - RNA, 21 nt, synthetic construct
  source 1..21: mol_type = other RNA
  misc_feature 20..21: note = T is dT
actgtcacaggaagaactttt

SEQ ID NO: 269 - RNA, 21 nt, synthetic construct
  source 1..21: mol_type = other RNA
  misc_feature 20..21: note = T is dT
ccgaacaagcaccgactgatt

SEQ ID NO: 270 - RNA, 21 nt, synthetic construct
  source 1..21: mol_type = other RNA
  misc_feature 20..21: note = T is dT
cctagaggctttttttgaatt

SEQ ID NO: 271 - RNA, 21 nt, synthetic construct
  source 1..21: mol_type = other RNA
  misc_feature 20..21: note = T is dT
caagcaccaactgagcaaatt

SEQ ID NO: 272 - RNA, 21 nt, synthetic construct
  source 1..21: mol_type = other RNA
  misc_feature 20..21: note = T is dT
ggacctgccaagcttggtctt

SEQ ID NO: 273 - RNA, 21 nt, synthetic construct
  source 1..21: mol_type = other RNA
  misc_feature 20..21: note = T is dT
accattatggacagagttatt

SEQ ID NO: 274 - RNA, 21 nt, synthetic construct
  source 1..21: mol_type = other RNA
  misc_feature 20..21: note = T is dT
gaagcaccaactgaaaacatt

SEQ ID NO: 275 - RNA, 21 nt, synthetic construct
  source 1..21: mol_type = other RNA
  misc_feature 20..21: note = T is dT
aggactgctactaccattatt

SEQ ID NO: 276 - RNA, 21 nt, synthetic construct
  source 1..21: mol_type = other RNA
  misc_feature 20..21: note = T is dT
ggctccttctgaacaagcatt

SEQ ID NO: 277 - RNA, 21 nt, synthetic construct
  source 1..21: mol_type = other RNA
  misc_feature 20..21: note = T is dT
aatccagatgctgagattatt

SEQ ID NO: 278 - RNA, 21 nt, synthetic construct
  source 1..21: mol_type = other RNA
  misc_feature 20..21: note = T is dT
cactatcacaggaagaacatt

SEQ ID NO: 279 - RNA, 21 nt, synthetic construct
  source 1..21: mol_type = other RNA
  misc_feature 20..21: note = T is dT
caagcaccgactgagcaaatt

SEQ ID NO: 280 - RNA, 21 nt, synthetic construct
  source 1..21: mol_type = other RNA
  misc_feature 20..21: note = T is dT
ggcacgtactccaccactgtt

SEQ ID NO: 281 - RNA, 21 nt, synthetic construct
  source 1..21: mol_type = other RNA
  misc_feature 20..21: note = T is dT
gctgagattcgcccttggttt

SEQ ID NO: 282 - RNA, 21 nt, synthetic construct
  source 1..21: mol_type = other RNA
  misc_feature 20..21: note = T is dT
ggctccttccgaacaagcatt

SEQ ID NO: 283 - RNA, 21 nt, synthetic construct
  source 1..21: mol_type = other RNA
  misc_feature 20..21: note = T is dT
agaagcaccaactgaaaactt

SEQ ID NO: 284 - RNA, 21 nt, synthetic construct
  source 1..21: mol_type = other RNA
  misc_feature 20..21: note = T is dT
ccttctgaagaagcaccaatt

SEQ ID NO: 285 - RNA, 21 nt, synthetic construct
  source 1..21: mol_type = other RNA
  misc_feature 20..21: note = T is dT
tgtggcagctccttattgttt

SEQ ID NO: 286 - RNA, 21 nt, synthetic construct
  source 1..21: mol_type = other RNA
  misc_feature 20..21: note = T is dT
gagttatcgaggctcattctt

SEQ ID NO: 287 - RNA, 21 nt, synthetic construct
  source 1..21: mol_type = other RNA
  misc_feature 20..21: note = T is dT
gaggctttttttgaacaagtt

SEQ ID NO: 288 - RNA, 21 nt, synthetic construct
  source 1..21: mol_type = other RNA
  misc_feature 20..21: note = T is dT
gcctagaggctccttctgatt

SEQ ID NO: 289 - RNA, 21 nt, synthetic construct
  source 1..21: mol_type = other RNA
  misc_feature 20..21: note = T is dT
aagaagcaccaactgaaaatt

SEQ ID NO: 290 - RNA, 21 nt, synthetic construct
  source 1..21: mol_type = other RNA
  misc_feature 20..21: note = T is dT
acaggaagaacatgtcagttt

SEQ ID NO: 291 - RNA, 21 nt, synthetic construct
  source 1..21: mol_type = other RNA
  misc_feature 20..21: note = T is dT
ggctgtttctgaacaagcatt

SEQ ID NO: 292 - RNA, 21 nt, synthetic construct
  source 1..21: mol_type = other RNA
  misc_feature 20..21: note = T is dT
cggtggtcccagttccaagtt

SEQ ID NO: 293 - RNA, 21 nt, synthetic construct
  source 1..21: mol_type = other RNA
  misc_feature 20..21: note = T is dT
aggacctgccaagcttggttt

SEQ ID NO: 294 - RNA, 21 nt, synthetic construct
  source 1..21: mol_type = other RNA
  misc_feature 20..21: note = T is dT
gtcgctcctccgactgtcatt

SEQ ID NO: 295 - RNA, 21 nt, synthetic construct
  source 1..21: mol_type = other RNA
  misc_feature 20..21: note = T is dT
caggactgctactaccatttt

SEQ ID NO: 296 - RNA, 21 nt, synthetic construct
  source 1..21: mol_type = other RNA
  misc_feature 20..21: note = T is dT
gcatcagaggacaacagaatt

SEQ ID NO: 297 - RNA, 21 nt, synthetic construct
  source 1..21: mol_type = other RNA
  misc_feature 20..21: note = T is dT
tggcttgatcaagaactactt

SEQ ID NO: 298 - RNA, 21 nt, synthetic construct
  source 1..21: mol_type = other RNA
  misc_feature 20..21: note = T is dT
cactggcatcagaggacaatt

SEQ ID NO: 299 - RNA, 21 nt, synthetic construct
  source 1..21: mol_type = other RNA
  misc_feature 20..21: note = T is dT
agcctagaggctccttctgtt

SEQ ID NO: 300 - RNA, 21 nt, synthetic construct
  source 1..21: mol_type = other RNA
  misc_feature 20..21: note = T is dT
gcacagaggcttcttctgatt

SEQ ID NO: 301 - RNA, 21 nt, synthetic construct
  source 1..21: mol_type = other RNA
  misc_feature 20..21: note = T is dT
cagaatcaggtgtcctagatt

SEQ ID NO: 302 - RNA, 21 nt, synthetic construct
  source 1..21: mol_type = other RNA
  misc_feature 20..21: note = T is dT
actatcacaggaagaacattt

SEQ ID NO: 303 - RNA, 21 nt, synthetic construct
  source 1..21: mol_type = other RNA
  misc_feature 20..21: note = T is dT
acaggactgctactaccattt

SEQ ID NO: 304 - RNA, 21 nt, synthetic construct
  source 1..21: mol_type = other RNA
  misc_feature 20..21: note = T is dT
ctaccattatggacagagttt

SEQ ID NO: 305 - RNA, 21 nt, synthetic construct
  source 1..21: mol_type = other RNA
  misc_feature 20..21: note = T is dT
gcctagaggctttttttgatt

SEQ ID NO: 306 - RNA, 21 nt, synthetic construct
  source 1..21: mol_type = other RNA
  misc_feature 20..21: note = T is dT
ccgccaggactgaatgttatt

SEQ ID NO: 307 - RNA, 21 nt, synthetic construct
  source 1..21: mol_type = other RNA
  misc_feature 20..21: note = T is dT
caagcaccaacggagcaaatt

SEQ ID NO: 308 - RNA, 21 nt, synthetic construct
  source 1..21: mol_type = other RNA
  misc_feature 20..21: note = T is dT
cccttggtgttacaccatgtt

SEQ ID NO: 309 - RNA, 21 nt, synthetic construct
  source 1..21: mol_type = other RNA
  misc_feature 20..21: note = T is dT
ctgctactaccattatggatt

SEQ ID NO: 310 - RNA, 21 nt, synthetic construct
  source 1..21: mol_type = other RNA
  misc_feature 20..21: note = T is dT
acaagcaccacctgagaaatt

SEQ ID NO: 311 - RNA, 21 nt, synthetic construct
  source 1..21: mol_type = other RNA
  misc_feature 20..21: note = T is dT
caatgcctggtgacagaattt

SEQ ID NO: 312 - RNA, 21 nt, synthetic construct
  source 1..21: mol_type = other RNA
  misc_feature 20..21: note = T is dT
aagcaccgactgagcaaagtt

SEQ ID NO: 313 - RNA, 21 nt, synthetic construct
  source 1..21: mol_type = other RNA
  misc_feature 20..21: note = T is dT
cacagaggcttcttctgaatt

SEQ ID NO: 314 - RNA, 21 nt, synthetic construct
  source 1..21: mol_type = other RNA
  misc_feature 20..21: note = T is dT
gtgtccttgcaactctcactt

SEQ ID NO: 315 - RNA, 21 nt, synthetic construct
  source 1..21: mol_type = other RNA
  misc_feature 20..21: note = T is dT
cagctccttattgttatactt

SEQ ID NO: 316 - RNA, 21 nt, synthetic construct
  source 1..21: mol_type = other RNA
  misc_feature 20..21: note = T is dT
gctccttccgaacaagcactt

SEQ ID NO: 317 - RNA, 21 nt, synthetic construct
  source 1..21: mol_type = other RNA
  misc_feature 20..21: note = T is dT
ggcatcagaggacaacagatt

SEQ ID NO: 318 - RNA, 21 nt, synthetic construct
  source 1..21: mol_type = other RNA
  misc_feature 20..21: note = T is dT
gcaccaactgaaaacagcatt

SEQ ID NO: 319 - RNA, 21 nt, synthetic construct
  source 1..21: mol_type = other RNA
  misc_feature 20..21: note = T is dT
tgctgagattcgcccttggtt

SEQ ID NO: 320 - RNA, 21 nt, synthetic construct
  source 1..21: mol_type = other RNA
  misc_feature 20..21: note = T is dT
ttccgaacaagcaccgacttt

SEQ ID NO: 321 - RNA, 21 nt, synthetic construct
  source 1..21: mol_type = other RNA
  misc_feature 20..21: note = T is dT
gctactaccattatggacatt

SEQ ID NO: 322 - RNA, 21 nt, synthetic construct
  source 1..21: mol_type = other RNA
  misc_feature 20..21: note = T is dT
gcaccaactgagcaaaggctt

SEQ ID NO: 323 - RNA, 21 nt, synthetic construct
  source 1..21: mol_type = other RNA
  misc_feature 20..21: note = T is dT
caggaagaacatgtcagtctt

SEQ ID NO: 324 - RNA, 21 nt, synthetic construct
  source 1..21: mol_type = other RNA
  misc_feature 20..21: note = T is dT
aagcaccaacggagcaaagtt

SEQ ID NO: 325 - RNA, 21 nt, synthetic construct
  source 1..21: mol_type = other RNA
  misc_feature 20..21: note = T is dT
gacaccacaccagcatagttt

SEQ ID NO: 326 - RNA, 21 nt, synthetic construct
  source 1..21: mol_type = other RNA
  misc_feature 20..21: note = T is dT
ctgtcacaggaagaacttgtt

SEQ ID NO: 327 - RNA, 21 nt, synthetic construct
  source 1..21: mol_type = other RNA
  misc_feature 20..21: note = T is dT
cagaggacaacagaatatttt

SEQ ID NO: 328 - RNA, 21 nt, synthetic construct
  source 1..21: mol_type = other RNA
  misc_feature 20..21: note = T is dT
ctggcatcagaggacaacatt

SEQ ID NO: 329 - RNA, 21 nt, synthetic construct
  source 1..21: mol_type = other RNA
  misc_feature 20..21: note = T is dT
taccattatggacagagtttt

SEQ ID NO: 330 - RNA, 21 nt, synthetic construct
  source 1..21: mol_type = other RNA
  misc_feature 20..21: note = T is dT
tcagaggacaacagaatattt

SEQ ID NO: 331 - RNA, 21 nt, synthetic construct
  source 1..21: mol_type = other RNA
  misc_feature 20..21: note = T is dT
catggatcccaatgtcagatt

SEQ ID NO: 332 - RNA, 21 nt, synthetic construct
  source 1..21: mol_type = other RNA
  misc_feature 20..21: note = T is dT
ccattatggacagagttactt

SEQ ID NO: 333 - RNA, 21 nt, synthetic construct
  source 1..21: mol_type = other RNA
  misc_feature 20..21: note = T is dT
ataccatggatcccaatgttt

SEQ ID NO: 334 - RNA, 21 nt, synthetic construct
  source 1..21: mol_type = other RNA
  misc_feature 20..21: note = T is dT
gctccttctgaacaagcactt

SEQ ID NO: 335 - RNA, 21 nt, synthetic construct
  source 1..21: mol_type = other RNA
  misc_feature 20..21: note = T is dT
gcaccgactgagcaaaggctt

SEQ ID NO: 336 - RNA, 21 nt, synthetic construct
  source 1..21: mol_type = other RNA
  misc_feature 20..21: note = T is dT
tccaagcctagaggctttttt

SEQ ID NO: 337 - RNA, 21 nt, synthetic construct
  source 1..21: mol_type = other RNA
  misc_feature 20..21: note = T is dT
tgacaccacaccagcatagtt

SEQ ID NO: 338 - RNA, 21 nt, synthetic construct
  source 1..21: mol_type = other RNA
  misc_feature 20..21: note = T is dT
cccagttccaagcacagagtt

SEQ ID NO: 339 - RNA, 21 nt, synthetic construct
  source 1..21: mol_type = other RNA
  misc_feature 20..21: note = T is dT
caccacaccagcatagtcgtt

SEQ ID NO: 340 - RNA, 21 nt, synthetic construct
  source 1..21: mol_type = other RNA
  misc_feature 20..21: note = T is dT
gtggtcccagttccaagcatt

SEQ ID NO: 341 - RNA, 21 nt, synthetic construct
  source 1..21: mol_type = other RNA
  misc_feature 20..21: note = T is dT
catcagaggacaacagaattt

SEQ ID NO: 342 - RNA, 21 nt, synthetic construct
  source 1..21: mol_type = other RNA
  misc_feature 20..21: note = T is dT
aagcacagaggcttcttcttt

SEQ ID NO: 343 - RNA, 21 nt, synthetic construct
  source 1..21: mol_type = other RNA
  misc_feature 20..21: note = T is dT
ggtggtcccagttccaagctt

SEQ ID NO: 344 - RNA, 21 nt, synthetic construct
  source 1..21: mol_type = other RNA
  misc_feature 20..21: note = T is dT
acaccacaccagcatagtctt

SEQ ID NO: 345 - RNA, 21 nt, synthetic construct
  source 1..21: mol_type = other RNA
  misc_feature 20..21: note = T is dT
agcaccgactgagcaaaggtt

SEQ ID NO: 346 - RNA, 21 nt, synthetic construct
  source 1..21: mol_type = other RNA
  misc_feature 20..21: note = T is dT
ctgacacgatgtccagtgatt

SEQ ID NO: 347 - RNA, 21 nt, synthetic construct
  source 1..21: mol_type = other RNA
  misc_feature 20..21: note = T is dT
gattcgcccttggtgttactt

SEQ ID NO: 348 - RNA, 21 nt, synthetic construct
  source 1..21: mol_type = other RNA
  misc_feature 20..21: note = T is dT
caccatggatcccagtgtctt

SEQ ID NO: 349 - RNA, 21 nt, synthetic construct
  source 1..21: mol_type = other RNA
  misc_feature 20..21: note = T is dT
ccaagcctagaggcttttttt

SEQ ID NO: 350 - RNA, 21 nt, synthetic construct
  source 1..21: mol_type = other RNA
  misc_feature 20..21: note = T is dT
agcacagaggcttcttctgtt

SEQ ID NO: 351 - RNA, 21 nt, synthetic construct
  source 1..21: mol_type = other RNA
  misc_feature 20..21: note = T is dT
cggctgtttctgaacaagctt

SEQ ID NO: 352 - RNA, 21 nt, synthetic construct
  source 1..21: mol_type = other RNA
  misc_feature 20..21: note = T is dT
gtggtcccagatccaagcatt

SEQ ID NO: 353 - RNA, 21 nt, synthetic construct
  source 1..21: mol_type = other RNA
  misc_feature 20..21: note = T is dT
ccagtgacagaatcgagtgtt

SEQ ID NO: 354 - RNA, 21 nt, synthetic construct
  source 1..21: mol_type = other RNA
  misc_feature 20..21: note = T is dT
atcagaggacaacagaatatt

SEQ ID NO: 355 - RNA, 21 nt, synthetic construct
  source 1..21: mol_type = other RNA
  misc_feature 20..21: note = T is dT
aagcaccaactgagcaaagtt

SEQ ID NO: 356 - RNA, 21 nt, synthetic construct
  source 1..21: mol_type = other RNA
  misc_feature 20..21: note = T is dT
gaagaacatgtcagtcttgtt

SEQ ID NO: 357 - RNA, 21 nt, synthetic construct
  source 1..21: mol_type = other RNA
  misc_feature 20..21: note = T is dT
aagcaccaactgaaaacagtt

SEQ ID NO: 358 - RNA, 21 nt, synthetic construct
  source 1..21: mol_type = other RNA
  misc_feature 20..21: note = T is dT
aggctccttctgaacaagctt

SEQ ID NO: 359 - RNA, 21 nt, synthetic construct
  source 1..21: mol_type = other RNA
  misc_feature 20..21: note = T is dT
agcaccaactgagcaaaggtt

SEQ ID NO: 360 - RNA, 21 nt, synthetic construct
  source 1..21: mol_type = other RNA
  misc_feature 20..21: note = T is dT
tcccacggtggtcccagtttt

SEQ ID NO: 361 - RNA, 21 nt, synthetic construct
  source 1..21: mol_type = other RNA
  misc_feature 20..21: note = T is dT
tccgaacaagcaccgactgtt

SEQ ID NO: 362 - RNA, 21 nt, synthetic construct
  source 1..21: mol_type = other RNA
  misc_feature 20..21: note = T is dT
tccacggctgtttctgaactt

SEQ ID NO: 363 - RNA, 21 nt, synthetic construct
  source 1..21: mol_type = other RNA
  misc_feature 20..21: note = T is dT
gaatcgagtgtcctcacaatt

SEQ ID NO: 364 - RNA, 21 nt, synthetic construct
  source 1..21: mol_type = other RNA
  misc_feature 20..21: note = T is dT
cctgacacgatgtccagtgtt

SEQ ID NO: 365 - RNA, 21 nt, synthetic construct
  source 1..21: mol_type = other RNA
  misc_feature 20..21: note = T is dT
tcctcacaactcccacggttt

SEQ ID NO: 366 - RNA, 21 nt, synthetic construct
  source 1..21: mol_type = other RNA
  misc_feature 20..21: note = T is dT
tggcatcagaggacaacagtt

SEQ ID NO: 367 - RNA, 21 nt, synthetic construct
  source 1..21: mol_type = other RNA
  misc_feature 20..21: note = T is dT
ggacaacagaatattatcctt

SEQ ID NO: 368 - RNA, 21 nt, synthetic construct
  source 1..21: mol_type = other RNA
  misc_feature 20..21: note = T is dT
ggtggtcccagatccaagctt

SEQ ID NO: 369 - RNA, 21 nt, synthetic construct
  source 1..21: mol_type = other RNA
  misc_feature 20..21: note = T is dT
aggcttcttctgaagaagctt

SEQ ID NO: 370 - RNA, 21 nt, synthetic construct
  source 1..21: mol_type = other RNA
  misc_feature 20..21: note = T is dT
tctcacggtggtcccagattt

SEQ ID NO: 371 - RNA, 21 nt, synthetic construct
  source 1..21: mol_type = other RNA
  misc_feature 20..21: note = T is dT
actggcatcagaggacaactt

SEQ ID NO: 372 - RNA, 21 nt, synthetic construct
  source 1..21: mol_type = other RNA
  misc_feature 20..21: note = T is dT
ggtgttataccatggatcctt

SEQ ID NO: 373 - RNA, 21 nt, synthetic construct
  source 1..21: mol_type = other RNA
  misc_feature 20..21: note = T is dT
acaccatggatcccagtgttt

SEQ ID NO: 374 - RNA, 21 nt, synthetic construct
  source 1..21: mol_type = other RNA
  misc_feature 20..21: note = T is dT
ctcacggtggtcccagatctt

SEQ ID NO: 375 - RNA, 21 nt, synthetic construct
  source 1..21: mol_type = other RNA
  misc_feature 20..21: note = T is dT
ccggttccaagcacagaggtt

SEQ ID NO: 376 - RNA, 21 nt, synthetic construct
  source 1..21: mol_type = other RNA
  misc_feature 20..21: note = T is dT
caagcacagaggcttcttctt

SEQ ID NO: 377 - RNA, 21 nt, synthetic construct
  source 1..21: mol_type = other RNA
  misc_feature 20..21: note = T is dT
cccttggtgttataccatgtt

SEQ ID NO: 378 - RNA, 21 nt, synthetic construct
  source 1..21: mol_type = other RNA
  misc_feature 20..21: note = T is dT
ttggtgttataccatggattt

SEQ ID NO: 379 - RNA, 21 nt, synthetic construct
  source 1..21: mol_type = other RNA
  misc_feature 20..21: note = T is dT
ggcttcttctgaagaagcatt

SEQ ID NO: 380 - RNA, 21 nt, synthetic construct
  source 1..21: mol_type = other RNA
  misc_feature 20..21: note = T is dT
aacaataaggagctgccactt

SEQ ID NO: 381 - RNA, 21 nt, synthetic construct
  source 1..21: mol_type = other RNA
  misc_feature 20..21: note = T is dT
tataacaataaggagctgctt

SEQ ID NO: 382 - RNA, 21 nt, synthetic construct
  source 1..21: mol_type = other RNA
  misc_feature 20..21: note = T is dT
ataacaataaggagctgcctt

SEQ ID NO: 383 - RNA, 21 nt, synthetic construct
  source 1..21: mol_type = other RNA
  misc_feature 20..21: note = T is dT
ttctgcgtctgagcattgctt

SEQ ID NO: 384 - RNA, 21 nt, synthetic construct
  source 1..21: mol_type = other RNA
  misc_feature 20..21: note = T is dT
cagtagttcttgatcaagctt

SEQ ID NO: 385 - RNA, 21 nt, synthetic construct
  source 1..21: mol_type = other RNA
  misc_feature 20..21: note = T is dT
ttcagaaggagcctctaggtt

SEQ ID NO: 386 - RNA, 21 nt, synthetic construct
  source 1..21: mol_type = other RNA
  misc_feature 20..21: note = T is dT
aaagcctctaggcttggagtt

SEQ ID NO: 387 - RNA, 21 nt, synthetic construct
  source 1..21: mol_type = other RNA
  misc_feature 20..21: note = T is dT
aagggcgaatctcagcatctt

SEQ ID NO: 388 - RNA, 21 nt, synthetic construct
  source 1..21: mol_type = other RNA
  misc_feature 20..21: note = T is dT
acagtggtggagtacgtgctt

SEQ ID NO: 389 - RNA, 21 nt, synthetic construct
  source 1..21: mol_type = other RNA
  misc_feature 20..21: note = T is dT
aatctcagcatctggattctt

SEQ ID NO: 390 - RNA, 21 nt, synthetic construct
  source 1..21: mol_type = other RNA
  misc_feature 20..21: note = T is dT
taacaataaggagctgccatt

SEQ ID NO: 391 - RNA, 21 nt, synthetic construct
  source 1..21: mol_type = other RNA
  misc_feature 20..21: note = T is dT
aatgagcctcgataactcttt

SEQ ID NO: 392 - RNA, 21 nt, synthetic construct
  source 1..21: mol_type = other RNA
  misc_feature 20..21: note = T is dT
ttggtgcttgttcagaaggtt

SEQ ID NO: 393 - RNA, 21 nt, synthetic construct
  source 1..21: mol_type = other RNA
  misc_feature 20..21: note = T is dT
aagttcttcctgtgacagttt

SEQ ID NO: 394 - RNA, 21 nt, synthetic construct
  source 1..21: mol_type = other RNA
  misc_feature 20..21: note = T is dT
tcagtcggtgcttgttcggtt

SEQ ID NO: 395 - RNA, 21 nt, synthetic construct
  source 1..21: mol_type = other RNA
  misc_feature 20..21: note = T is dT
ttcaaaaaaagcctctaggtt

SEQ ID NO: 396 - RNA, 21 nt, synthetic construct
  source 1..21: mol_type = other RNA
  misc_feature 20..21: note = T is dT
tttgctcagttggtgcttgtt

SEQ ID NO: 397 - RNA, 21 nt, synthetic construct
  source 1..21: mol_type = other RNA
  misc_feature 20..21: note = T is dT
gaccaagcttggcaggtcctt

SEQ ID NO: 398 - RNA, 21 nt, synthetic construct
  source 1..21: mol_type = other RNA
  misc_feature 20..21: note = T is dT
taactctgtccataatggttt

SEQ ID NO: 399 - RNA, 21 nt, synthetic construct
  source 1..21: mol_type = other RNA
  misc_feature 20..21: note = T is dT
tgttttcagttggtgcttctt

SEQ ID NO: 400 - RNA, 21 nt, synthetic construct
  source 1..21: mol_type = other RNA
  misc_feature 20..21: note = T is dT
taatggtagtagcagtccttt

SEQ ID NO: 401 - RNA, 21 nt, synthetic construct
  source 1..21: mol_type = other RNA
  misc_feature 20..21: note = T is dT
tgcttgttcagaaggagcctt

SEQ ID NO: 402 - RNA, 21 nt, synthetic construct
  source 1..21: mol_type = other RNA
  misc_feature 20..21: note = T is dT
taatctcagcatctggatttt

SEQ ID NO: 403 - RNA, 21 nt, synthetic construct
  source 1..21: mol_type = other RNA
  misc_feature 20..21: note = T is dT
tgttcttcctgtgatagtgtt

SEQ ID NO: 404 - RNA, 21 nt, synthetic construct
  source 1..21: mol_type = other RNA
  misc_feature 20..21: note = T is dT
tttgctcagtcggtgcttgtt

SEQ ID NO: 405 - RNA, 21 nt, synthetic construct
  source 1..21: mol_type = other RNA
  misc_feature 20..21: note = T is dT
cagtggtggagtacgtgcctt

SEQ ID NO: 406 - RNA, 21 nt, synthetic construct
  source 1..21: mol_type = other RNA
  misc_feature 20..21: note = T is dT
accaagggcgaatctcagctt

SEQ ID NO: 407 - RNA, 21 nt, synthetic construct
  source 1..21: mol_type = other RNA
  misc_feature 20..21: note = T is dT
tgcttgttcggaaggagcctt

SEQ ID NO: 408 - RNA, 21 nt, synthetic construct
  source 1..21: mol_type = other RNA
  misc_feature 20..21: note = T is dT
gttttcagttggtgcttcttt

SEQ ID NO: 409 - RNA, 21 nt, synthetic construct
  source 1..21: mol_type = other RNA
  misc_feature 20..21: note = T is dT
ttggtgcttcttcagaaggtt

SEQ ID NO: 410 - RNA, 21 nt, synthetic construct
  source 1..21: mol_type = other RNA
  misc_feature 20..21: note = T is dT
acaataaggagctgccacatt

SEQ ID NO: 411 - RNA, 21 nt, synthetic construct
  source 1..21: mol_type = other RNA
  misc_feature 20..21: note = T is dT
gaatgagcctcgataactctt

SEQ ID NO: 412 - RNA, 21 nt, synthetic construct
  source 1..21: mol_type = other RNA
  misc_feature 20..21: note = T is dT
cttgttcaaaaaaagcctctt

SEQ ID NO: 413 - RNA, 21 nt, synthetic construct
  source 1..21: mol_type = other RNA
  misc_feature 20..21: note = T is dT
tcagaaggagcctctaggctt

SEQ ID NO: 414 - RNA, 21 nt, synthetic construct
  source 1..21: mol_type = other RNA
  misc_feature 20..21: note = T is dT
ttttcagttggtgcttctttt

SEQ ID NO: 415 - RNA, 21 nt, synthetic construct
  source 1..21: mol_type = other RNA
  misc_feature 20..21: note = T is dT
actgacatgttcttcctgttt

SEQ ID NO: 416 - RNA, 21 nt, synthetic construct
  source 1..21: mol_type = other RNA
  misc_feature 20..21: note = T is dT
tgcttgttcagaaacagcctt

SEQ ID NO: 417 - RNA, 21 nt, synthetic construct
  source 1..21: mol_type = other RNA
  misc_feature 20..21: note = T is dT
cttggaactgggaccaccgtt

SEQ ID NO: 418 - RNA, 21 nt, synthetic construct
  source 1..21: mol_type = other RNA
  misc_feature 20..21: note = T is dT
accaagcttggcaggtccttt

SEQ ID NO: 419 - RNA, 21 nt, synthetic construct
  source 1..21: mol_type = other RNA
  misc_feature 20..21: note = T is dT
tgacagtcggaggagcgactt

SEQ ID NO: 420 - RNA, 21 nt, synthetic construct
  source 1..21: mol_type = other RNA
  misc_feature 20..21: note = T is dT
aatggtagtagcagtcctgtt

SEQ ID NO: 421 - RNA, 21 nt, synthetic construct
  source 1..21: mol_type = other RNA
  misc_feature 20..21: note = T is dT
ttctgttgtcctctgatgctt

SEQ ID NO: 422 - RNA, 21 nt, synthetic construct
  source 1..21: mol_type = other RNA
  misc_feature 20..21: note = T is dT
gtagttcttgatcaagccatt

SEQ ID NO: 423 - RNA, 21 nt, synthetic construct
  source 1..21: mol_type = other RNA
  misc_feature 20..21: note = T is dT
ttgtcctctgatgccagtgtt

SEQ ID NO: 424 - RNA, 21 nt, synthetic construct
  source 1..21: mol_type = other RNA
  misc_feature 20..21: note = T is dT
cagaaggagcctctaggcttt

SEQ ID NO: 425 - RNA, 21 nt, synthetic construct
  source 1..21: mol_type = other RNA
  misc_feature 20..21: note = T is dT
tcagaagaagcctctgtgctt

SEQ ID NO: 426 - RNA, 21 nt, synthetic construct
  source 1..21: mol_type = other RNA
  misc_feature 20..21: note = T is dT
tctaggacacctgattctgtt

SEQ ID NO: 427 - RNA, 21 nt, synthetic construct
  source 1..21: mol_type = other RNA
  misc_feature 20..21: note = T is dT
atgttcttcctgtgatagttt

SEQ ID NO: 428 - RNA, 21 nt, synthetic construct
  source 1..21: mol_type = other RNA
  misc_feature 20..21: note = T is dT
atggtagtagcagtcctgttt

SEQ ID NO: 429 - RNA, 21 nt, synthetic construct
  source 1..21: mol_type = other RNA
  misc_feature 20..21: note = T is dT
actctgtccataatggtagtt

SEQ ID NO: 430 - RNA, 21 nt, synthetic construct
  source 1..21: mol_type = other RNA
  misc_feature 20..21: note = T is dT
tcaaaaaaagcctctaggctt

SEQ ID NO: 431 - RNA, 21 nt, synthetic construct
  source 1..21: mol_type = other RNA
  misc_feature 20..21: note = T is dT
taacattcagtcctggcggtt

SEQ ID NO: 432 - RNA, 21 nt, synthetic construct
  source 1..21: mol_type = other RNA
  misc_feature 20..21: note = T is dT
tttgctccgttggtgcttgtt

SEQ ID NO: 433 - RNA, 21 nt, synthetic construct
  source 1..21: mol_type = other RNA
  misc_feature 20..21: note = T is dT
catggtgtaacaccaagggtt

SEQ ID NO: 434 - RNA, 21 nt, synthetic construct
  source 1..21: mol_type = other RNA
  misc_feature 20..21: note = T is dT
tccataatggtagtagcagtt

SEQ ID NO: 435 - RNA, 21 nt, synthetic construct
  source 1..21: mol_type = other RNA
  misc_feature 20..21: note = T is dT
tttctcaggtggtgcttgttt

SEQ ID NO: 436 - RNA, 21 nt, synthetic construct
  source 1..21: mol_type = other RNA
  misc_feature 20..21: note = T is dT
attctgtcaccaggcattgtt

SEQ ID NO: 437 - RNA, 21 nt, synthetic construct
  source 1..21: mol_type = other RNA
  misc_feature 20..21: note = T is dT
ctttgctcagtcggtgctttt

SEQ ID NO: 438 - RNA, 21 nt, synthetic construct
  source 1..21: mol_type = other RNA
  misc_feature 20..21: note = T is dT
ttcagaagaagcctctgtgtt

SEQ ID NO: 439 - RNA, 21 nt, synthetic construct
  source 1..21: mol_type = other RNA
  misc_feature 20..21: note = T is dT
gtgagagttgcaaggacactt

SEQ ID NO: 440 - RNA, 21 nt, synthetic construct
  source 1..21: mol_type = other RNA
  misc_feature 20..21: note = T is dT
gtataacaataaggagctgtt

SEQ ID NO: 441 - RNA, 21 nt, synthetic construct
  source 1..21: mol_type = other RNA
  misc_feature 20..21: note = T is dT
gtgcttgttcggaaggagctt

SEQ ID NO: 442 - RNA, 21 nt, synthetic construct
  source 1..21: mol_type = other RNA
  misc_feature 20..21: note = T is dT
tctgttgtcctctgatgcctt

SEQ ID NO: 443 - RNA, 21 nt, synthetic construct
  source 1..21: mol_type = other RNA
  misc_feature 20..21: note = T is dT
tgctgttttcagttggtgctt

SEQ ID NO: 444 - RNA, 21 nt, synthetic construct
  source 1..21: mol_type = other RNA
  misc_feature 20..21: note = T is dT
ccaagggcgaatctcagcatt

SEQ ID NO: 445 - RNA, 21 nt, synthetic construct
  source 1..21: mol_type = other RNA
  misc_feature 20..21: note = T is dT
agtcggtgcttgttcggaatt

SEQ ID NO: 446 - RNA, 21 nt, synthetic construct
  source 1..21: mol_type = other RNA
  misc_feature 20..21: note = T is dT
tgtccataatggtagtagctt

SEQ ID NO: 447 - RNA, 21 nt, synthetic construct
  source 1..21: mol_type = other RNA
  misc_feature 20..21: note = T is dT
gcctttgctcagttggtgctt

SEQ ID NO: 448 - RNA, 21 nt, synthetic construct
  source 1..21: mol_type = other RNA
  misc_feature 20..21: note = T is dT
gactgacatgttcttcctgtt

SEQ ID NO: 449 - RNA, 21 nt, synthetic construct
  source 1..21: mol_type = other RNA
  misc_feature 20..21: note = T is dT
ctttgctccgttggtgctttt

SEQ ID NO: 450 - RNA, 21 nt, synthetic construct
  source 1..21: mol_type = other RNA
  misc_feature 20..21: note = T is dT
actatgctggtgtggtgtctt

SEQ ID NO: 451 - RNA, 21 nt, synthetic construct
  source 1..21: mol_type = other RNA
  misc_feature 20..21: note = T is dT
caagttcttcctgtgacagtt

SEQ ID NO: 452 - RNA, 21 nt, synthetic construct
  source 1..21: mol_type = other RNA
  misc_feature 20..21: note = T is dT
aatattctgttgtcctctgtt

SEQ ID NO: 453 - RNA, 21 nt, synthetic construct
  source 1..21: mol_type = other RNA
  misc_feature 20..21: note = T is dT
tgttgtcctctgatgccagtt

SEQ ID NO: 454 - RNA, 21 nt, synthetic construct
  source 1..21: mol_type = other RNA
  misc_feature 20..21: note = T is dT
aactctgtccataatggtatt

SEQ ID NO: 455 - RNA, 21 nt, synthetic construct
  source 1..21: mol_type = other RNA
  misc_feature 20..21: note = T is dT
atattctgttgtcctctgatt

SEQ ID NO: 456 - RNA, 21 nt, synthetic construct
  source 1..21: mol_type = other RNA
  misc_feature 20..21: note = T is dT
tctgacattgggatccatgtt

SEQ ID NO: 457 - RNA, 21 nt, synthetic construct
  source 1..21: mol_type = other RNA
  misc_feature 20..21: note = T is dT
gtaactctgtccataatggtt

SEQ ID NO: 458 - RNA, 21 nt, synthetic construct
  source 1..21: mol_type = other RNA
  misc_feature 20..21: note = T is dT
acattgggatccatggtattt

SEQ ID NO: 459 - RNA, 21 nt, synthetic construct
  source 1..21: mol_type = other RNA
  misc_feature 20..21: note = T is dT
gtgcttgttcagaaggagctt

SEQ ID NO: 460 - RNA, 21 nt, synthetic construct
  source 1..21: mol_type = other RNA
  misc_feature 20..21: note = T is dT
gcctttgctcagtcggtgctt

SEQ ID NO: 461 - RNA, 21 nt, synthetic construct
  source 1..21: mol_type = other RNA
  misc_feature 20..21: note = T is dT
aaaagcctctaggcttggatt

SEQ ID NO: 462 - RNA, 21 nt, synthetic construct
  source 1..21: mol_type = other RNA
  misc_feature 20..21: note = T is dT
ctatgctggtgtggtgtcatt

SEQ ID NO: 463 - RNA, 21 nt, synthetic construct
  source 1..21: mol_type = other RNA
  misc_feature 20..21: note = T is dT
ctctgtgcttggaactgggtt

SEQ ID NO: 464 - RNA, 21 nt, synthetic construct
  source 1..21: mol_type = other RNA
  misc_feature 20..21: note = T is dT
cgactatgctggtgtggtgtt

SEQ ID NO: 465 - RNA, 21 nt, synthetic construct
  source 1..21: mol_type = other RNA
  misc_feature 20..21: note = T is dT
tgcttggaactgggaccactt

SEQ ID NO: 466 - RNA, 21 nt, synthetic construct
  source 1..21: mol_type = other RNA
  misc_feature 20..21: note = T is dT
attctgttgtcctctgatgtt

SEQ ID NO: 467 - RNA, 21 nt, synthetic construct
  source 1..21: mol_type = other RNA
  misc_feature 20..21: note = T is dT
agaagaagcctctgtgctttt

SEQ ID NO: 468 - RNA, 21 nt, synthetic construct
  source 1..21: mol_type = other RNA
  misc_feature 20..21: note = T is dT
gcttggaactgggaccacctt

SEQ ID NO: 469 - RNA, 21 nt, synthetic construct
  source 1..21: mol_type = other RNA
  misc_feature 20..21: note = T is dT
gactatgctggtgtggtgttt

SEQ ID NO: 470 - RNA, 21 nt, synthetic construct
  source 1..21: mol_type = other RNA
  misc_feature 20..21: note = T is dT
cctttgctcagtcggtgcttt

SEQ ID NO: 471 - RNA, 21 nt, synthetic construct
  source 1..21: mol_type = other RNA
  misc_feature 20..21: note = T is dT
tcactggacatcgtgtcagtt

SEQ ID NO: 472 - RNA, 21 nt, synthetic construct
  source 1..21: mol_type = other RNA
  misc_feature 20..21: note = T is dT
gtaacaccaagggcgaatctt

SEQ ID NO: 473 - RNA, 21 nt, synthetic construct
  source 1..21: mol_type = other RNA
  misc_feature 20..21: note = T is dT
gacactgggatccatggtgtt

SEQ ID NO: 474 - RNA, 21 nt, synthetic construct
  source 1..21: mol_type = other RNA
  misc_feature 20..21: note = T is dT
aaaaagcctctaggcttggtt

SEQ ID NO: 475 - RNA, 21 nt, synthetic construct
  source 1..21: mol_type = other RNA
  misc_feature 20..21: note = T is dT
cagaagaagcctctgtgcttt

SEQ ID NO: 476 - RNA, 21 nt, synthetic construct
  source 1..21: mol_type = other RNA
  misc_feature 20..21: note = T is dT
gcttgttcagaaacagccgtt

SEQ ID NO: 477 - RNA, 21 nt, synthetic construct
  source 1..21: mol_type = other RNA
  misc_feature 20..21: note = T is dT
tgcttggatctgggaccactt

SEQ ID NO: 478 - RNA, 21 nt, synthetic construct
  source 1..21: mol_type = other RNA
  misc_feature 20..21: note = T is dT
cactcgattctgtcactggtt

SEQ ID NO: 479 - RNA, 21 nt, synthetic construct
  source 1..21: mol_type = other RNA
  misc_feature 20..21: note = T is dT
tattctgttgtcctctgattt

SEQ ID NO: 480 - RNA, 21 nt, synthetic construct
  source 1..21: mol_type = other RNA
  misc_feature 20..21: note = T is dT
ctttgctcagttggtgctttt

SEQ ID NO: 481 - RNA, 21 nt, synthetic construct
  source 1..21: mol_type = other RNA
  misc_feature 20..21: note = T is dT
caagactgacatgttcttctt

SEQ ID NO: 482 - RNA, 21 nt, synthetic construct
  source 1..21: mol_type = other RNA
  misc_feature 20..21: note = T is dT
ctgttttcagttggtgctttt

SEQ ID NO: 483 - RNA, 21 nt, synthetic construct
  source 1..21: mol_type = other RNA
  misc_feature 20..21: note = T is dT
gcttgttcagaaggagccttt

SEQ ID NO: 484 - RNA, 21 nt, synthetic construct
  source 1..21: mol_type = other RNA
  misc_feature 20..21: note = T is dT
cctttgctcagttggtgcttt

SEQ ID NO: 485 - RNA, 21 nt, synthetic construct
  source 1..21: mol_type = other RNA
  misc_feature 20..21: note = T is dT
aactgggaccaccgtgggatt

SEQ ID NO: 486 - RNA, 21 nt, synthetic construct
  source 1..21: mol_type = other RNA
  misc_feature 20..21: note = T is dT
cagtcggtgcttgttcggatt

SEQ ID NO: 487 - RNA, 21 nt, synthetic construct
  source 1..21: mol_type = other RNA
  misc_feature 20..21: note = T is dT
gttcagaaacagccgtggatt

SEQ ID NO: 488 - RNA, 21 nt, synthetic construct
  source 1..21: mol_type = other RNA
  misc_feature 20..21: note = T is dT
ttgtgaggacactcgattctt

SEQ ID NO: 489 - RNA, 21 nt, synthetic construct
  source 1..21: mol_type = other RNA
  misc_feature 20..21: note = T is dT
cactggacatcgtgtcaggtt

SEQ ID NO: 490 - RNA, 21 nt, synthetic construct
  source 1..21: mol_type = other RNA
  misc_feature 20..21: note = T is dT
accgtgggagttgtgaggatt

SEQ ID NO: 491 - RNA, 21 nt, synthetic construct
  source 1..21: mol_type = other RNA
  misc_feature 20..21: note = T is dT
ctgttgtcctctgatgccatt

SEQ ID NO: 492 - RNA, 21 nt, synthetic construct
  source 1..21: mol_type = other RNA
  misc_feature 20..21: note = T is dT
ggataatattctgttgtcctt

SEQ ID NO: 493 - RNA, 21 nt, synthetic construct
  source 1..21: mol_type = other RNA
  misc_feature 20..21: note = T is dT
gcttggatctgggaccacctt

SEQ ID NO: 494 - RNA, 21 nt, synthetic construct
  source 1..21: mol_type = other RNA
  misc_feature 20..21: note = T is dT
gcttcttcagaagaagccttt

SEQ ID NO: 495 - RNA, 21 nt, synthetic construct
  source 1..21: mol_type = other RNA
  misc_feature 20..21: note = T is dT
atctgggaccaccgtgagatt

SEQ ID NO: 496 - RNA, 21 nt, synthetic construct
  source 1..21: mol_type = other RNA
  misc_feature 20..21: note = T is dT
gttgtcctctgatgccagttt

SEQ ID NO: 497 - RNA, 21 nt, synthetic construct
  source 1..21: mol_type = other RNA
  misc_feature 20..21: note = T is dT
ggatccatggtataacacctt

SEQ ID NO: 498 - RNA, 21 nt, synthetic construct
  source 1..21: mol_type = other RNA
  misc_feature 20..21: note = T is dT
acactgggatccatggtgttt

SEQ ID NO: 499 - RNA, 21 nt, synthetic construct
  source 1..21: mol_type = other RNA
  misc_feature 20..21: note = T is dT
gatctgggaccaccgtgagtt

SEQ ID NO: 500 - RNA, 21 nt, synthetic construct
  source 1..21: mol_type = other RNA
  misc_feature 20..21: note = T is dT
cctctgtgcttggaaccggtt

SEQ ID NO: 501 - RNA, 21 nt, synthetic construct
  source 1..21: mol_type = other RNA
  misc_feature 20..21: note = T is dT
gaagaagcctctgtgcttgtt

SEQ ID NO: 502 - RNA, 21 nt, synthetic construct
  source 1..21: mol_type = other RNA
  misc_feature 20..21: note = T is dT
catggtataacaccaagggtt

SEQ ID NO: 503 - RNA, 21 nt, synthetic construct
  source 1..21: mol_type = other RNA
  misc_feature 20..21: note = T is dT
atccatggtataacaccaatt

SEQ ID NO: 504 - RNA, 21 nt, synthetic construct
  source 1..21: mol_type = other RNA
  misc_feature 20..21: note = T is dT
tgcttcttcagaagaagcctt

SEQ ID NO: 505 - RNA, 23 nt, synthetic construct
  source 1..23: mol_type = other RNA
  misc_feature 1..3: note = modified _base - linked via monothioate phosphorodiester bond
  misc_feature 21..23: note = modified _base - linked via monothioate phosphorodiester bond
  misc_feature 1..23: note = 2'-OH of the nucleotides at positions 2,6,14,16 from the 5' end is replaced by fluorine, 2'-OH of the remaining nucleotides is replaced by methoxy group.
tataacaataaggagctgccaca

SEQ ID NO: 506 - RNA, 21 nt, synthetic construct
  source 1..21: mol_type = other RNA
  misc_feature 1..3: note = modified _base - linked via monothioate phosphorodiester bond
  misc_feature 19..21: note = modified _base - linked via monothioate phosphorodiester bond
  misc_feature 1..21: note = 2'-OH of the nucleotides at positions 9,10,11, from the 5' end is replaced by fluorine, 2'-OH of the remaining nucleotides is replaced by methoxy group.
tggcagctccttattgttata

SEQ ID NO: 507 - RNA, 21 nt, synthetic construct
  source 1..21: mol_type = other RNA
  misc_feature 20..21: note = T is dT
  misc_feature 1..3: note = modified _base - linked via monothioate phosphorodiester bond
  misc_feature 19..21: note = modified _base - linked via monothioate phosphorodiester bond
  misc_feature 1..19: note = 2'-OH of the nucleotides at positions 2,6,8,14,16 from the 5' end is replaced by fluorine, 2'-OH of the remaining nucleotides is replaced by methoxy group.
tataacaataaggagctgctt

SEQ ID NO: 508 - RNA, 19 nt, synthetic construct
  source 1..19: mol_type = other RNA
  misc_feature 1..3: note = modified _base - linked via monothioate phosphorodiester bond
  misc_feature 17..19: note = modified _base - linked via monothioate phosphorodiester bond
  misc_feature 1..19: note = 2'-OH of the nucleotides at positions 7,8,9 from the 5' end is replaced by fluorine, 2'-OH of the remaining nucleotides is replaced by methoxy group.
gcagctccttattgttata

SEQ ID NO: 509 - RNA, 21 nt, synthetic construct
  source 1..21: mol_type = other RNA
  misc_feature 20..21: note = T is dT
  misc_feature 1..3: note = modified _base - linked via monothioate phosphorodiester bond
  misc_feature 19..21: note = modified _base - linked via monothioate phosphorodiester bond
  misc_feature 1..19: note = 2'-OH of the nucleotides at positions 2,6,8,14,16 from the 5' end is replaced by fluorine, 2'-OH of the remaining nucleotides is replaced by methoxy group.
tataacaataaggagctgctt

SEQ ID NO: 510 - RNA, 19 nt, synthetic construct
  source 1..19: mol_type = other RNA
  misc_feature 1..3: note = modified _base - linked via monothioate phosphorodiester bond
  misc_feature 17..19: note = modified _base - linked via monothioate phosphorodiester bond
  misc_feature 1..19: note = 2'-OH of the nucleotides at positions 7,8,9 from the 5' end is replaced by fluorine, 2'-OH of the remaining nucleotides is replaced by methoxy group.
gcagctccttattgttata

SEQ ID NO: 511 - RNA, 21 nt, synthetic construct
  source 1..21: mol_type = other RNA
  misc_feature 20..21: note = T is dT
  misc_feature 1..3: note = modified _base - linked via monothioate phosphorodiester bond
  misc_structure 1: note = modified with 5'-(E)-vinylphosphonate group
  misc_feature 19..21: note = modified _base - linked via monothioate phosphorodiester bond
  misc_feature 1..19: note = 2'-OH of the nucleotides at positions 2,6,8,14,16 from the 5' end is replaced by fluorine, 2'-OH of the remaining nucleotides is replaced by methoxy group.
tataacaataaggagctgctt

SEQ ID NO: 512 - RNA, 19 nt, synthetic construct
  source 1..19: mol_type = other RNA
  misc_feature 1..3: note = modified _base - linked via monothioate phosphorodiester bond
  misc_feature 17..19: note = modified _base - linked via monothioate phosphorodiester bond
  misc_feature 1..19: note = 2'-OH of the nucleotides at positions 7,8,9 from the 5' end is replaced by fluorine, 2'-OH of the remaining nucleotides is replaced by methoxy group.
gcagctccttattgttata

SEQ ID NO: 513 - RNA, 21 nt, synthetic construct
  source 1..21: mol_type = other RNA
  misc_feature 20..21: note = T is dT
  misc_feature 1..3: note = modified _base - linked via monothioate phosphorodiester bond
  misc_feature 1: note = modified with 5'-(E)-vinylphosphonate group
  misc_feature 19..21: note = modified _base - linked via monothioate phosphorodiester bond
  misc_feature 1..19: note = 2'-OH of the nucleotides at positions 2,6,8,14,16 from the 5' end is replaced by fluorine, 2'-OH of the remaining nucleotides is replaced by methoxy group.
tataacaataaggagctgctt

SEQ ID NO: 514 - RNA, 19 nt, synthetic construct
  source 1..19: mol_type = other RNA
  misc_feature 1..3: note = modified _base - linked via monothioate phosphorodiester bond
  misc_feature 17..19: note = modified _base - linked via monothioate phosphorodiester bond
  misc_feature 1..19: note = 2'-OH of the nucleotides at positions 7,8,9 from the 5' end is replaced by fluorine, 2'-OH of the remaining nucleotides is replaced by methoxy group.
gcagctccttattgttata

SEQ ID NO: 515 - RNA, 21 nt, synthetic construct
  source 1..21: mol_type = other RNA
  misc_feature 20..21: note = T is dT
  misc_feature 1..3: note = modified _base - linked via monothioate phosphorodiester bond
  misc_feature 19..21: note = modified _base - linked via monothioate phosphorodiester bond
  misc_feature 1..19: note = 2'-OH of the nucleotides at positions 2,6,8,14,16 from the 5' end is replaced by fluorine, 2'-OH of the remaining nucleotides is replaced by methoxy group.
cagtagttcttgatcaagctt

SEQ ID NO: 516 - RNA, 19 nt, synthetic construct
  source 1..19: mol_type = other RNA
  misc_feature 1..3: note = modified _base - linked via monothioate phosphorodiester bond
  misc_feature 17..19: note = modified _base - linked via monothioate phosphorodiester bond
  misc_feature 1..19: note = 2'-OH of the nucleotides at positions 7,8,9 from the 5' end is replaced by fluorine, 2'-OH of the remaining nucleotides is replaced by methoxy group.
gcttgatcaagaactactg

SEQ ID NO: 517 - RNA, 21 nt, synthetic construct
  source 1..21: mol_type = other RNA
  misc_feature 20..21: note = T is dT
  misc_feature 1..3: note = modified _base - linked via monothioate phosphorodiester bond
  misc_feature 19..21: note = modified _base - linked via monothioate phosphorodiester bond
  misc_feature 1..19: note = 2'-OH of the nucleotides at positions 2,6,8,14,16 from the 5' end is replaced by fluorine, 2'-OH of the remaining nucleotides is replaced by methoxy group.
aacaataaggagctgccactt

SEQ ID NO: 518 - RNA, 19 nt, synthetic construct
  source 1..19: mol_type = other RNA
  misc_feature 1..3: note = modified _base - linked via monothioate phosphorodiester bond
  misc_feature 17..19: note = modified _base - linked via monothioate phosphorodiester bond
  misc_feature 1..19: note = 2'-OH of the nucleotides at positions 7,8,9 from the 5' end is replaced by fluorine, 2'-OH of the remaining nucleotides is replaced by methoxy group.
gtggcagctccttattgtt

SEQ ID NO: 519 - RNA, 21 nt, synthetic construct
  source 1..21: mol_type = other RNA
  misc_feature 20..21: note = T is dT
  misc_feature 1..3: note = modified _base - linked via monothioate phosphorodiester bond
  misc_feature 19..21: note = modified _base - linked via monothioate phosphorodiester bond
  misc_feature 1..19: note = 2'-OH of the nucleotides at positions 2,6,14,16 from the 5' end is replaced by fluorine, 2'-OH of the remaining nucleotides is replaced by methoxy group.
tataacaataaggagctgctt

SEQ ID NO: 520 - RNA, 19 nt, synthetic construct
  source 1..19: mol_type = other RNA
  misc_feature 1..3: note = modified _base - linked via monothioate phosphorodiester bond
  misc_feature 17..19: note = modified _base - linked via monothioate phosphorodiester bond
  misc_feature 1..19: note = 2'-OH of the nucleotides at positions 7,8,9 from the 5' end is replaced by fluorine, 2'-OH of the remaining nucleotides is replaced by methoxy group.
gcagctccttattgttata

SEQ ID NO: 521 - RNA, 21 nt, synthetic construct
  source 1..21: mol_type = other RNA
  misc_feature 1..3: note = modified _base - linked via monothioate phosphorodiester bond
  misc_feature 19..21: note = modified _base - linked via monothioate phosphorodiester bond
  misc_feature 1..21: note = 2'-OH of the nucleotides at positions 2,4,6,12,14,16 from the 5' end is replaced by fluorine, 2'-OH of the remaining nucleotides is replaced by methoxy group.
aatgagcctcgataactctgt

SEQ ID NO: 522 - RNA, 21 nt, synthetic construct
  source 1..21: mol_type = other RNA
  misc_feature 1..3: note = modified _base - linked via monothioate phosphorodiester bond
  misc_feature 19..21: note = modified _base - linked via monothioate phosphorodiester bond
  misc_feature 1..21: note = 2'-OH of the nucleotides at positions 9,10,11 from the 5' end is replaced by fluorine, 2'-OH of the remaining nucleotides is replaced by methoxy group.
acagagttatcgaggctcatt

SEQ ID NO: 523 - RNA, 21 nt, synthetic construct
  source 1..21: mol_type = other RNA
  misc_feature 1..3: note = modified _base - linked via monothioate phosphorodiester bond
  misc_feature 19..21: note = modified _base - linked via monothioate phosphorodiester bond
  misc_feature 1..21: note = 2'-OH of the nucleotides at positions 2,4,6,12,14,16 from the 5' end is replaced by fluorine, 2'-OH of the remaining nucleotides is replaced by methoxy group.
aagggcgaatctcagcatctg

SEQ ID NO: 524 - RNA, 21 nt, synthetic construct
  source 1..21: mol_type = other RNA
  misc_feature 1..3: note = modified _base - linked via monothioate phosphorodiester bond
  misc_feature 19..21: note = modified _base - linked via monothioate phosphorodiester bond
  misc_feature 1..21: note = 2'-OH of the nucleotides at positions 9,10,11 from the 5' end is replaced by fluorine, 2'-OH of the remaining nucleotides is replaced by methoxy group.
cagatgctgagattcgccctt

SEQ ID NO: 525 - RNA, 21 nt, synthetic construct
  source 1..21: mol_type = other RNA
  misc_feature 1..3: note = modified _base - linked via monothioate phosphorodiester bond
  misc_feature 1: note = modified with 5'-(E)-vinylphosphonate group
  misc_feature 19..21: note = modified _base - linked via monothioate phosphorodiester bond
  misc_feature 1..21: note = 2'-OH of the nucleotides at positions 2,4,6,12,14,16 from the 5' end is replaced by fluorine, 2'-OH of the remaining nucleotides is replaced by methoxy group.
aagggcgaatctcagcatctg

SEQ ID NO: 526 - RNA, 21 nt, synthetic construct
  source 1..21: mol_type = other RNA
  misc_feature 1..3: note = modified _base - linked via monothioate phosphorodiester bond
  misc_feature 19..21: note = modified _base - linked via monothioate phosphorodiester bond
  misc_feature 1..21: note = 2'-OH of the nucleotides at positions 9,10,11 from the 5' end is replaced by fluorine, 2'-OH of the remaining nucleotides is replaced by methoxy group.
cagatgctgagattcgccctt

SEQ ID NO: 527 - RNA, 21 nt, synthetic construct
  source 1..21: mol_type = other RNA
  misc_feature 1..3: note = modified _base - linked via monothioate phosphorodiester bond
  misc_feature 1: note = modified with 5'-(E)-vinylphosphonate group
  misc_feature 19..21: note = modified _base - linked via monothioate phosphorodiester bond
  misc_feature 1..21: note = 2'-OH of the nucleotides at positions 2,4,6,12,14,16 from the 5' end is replaced by fluorine, 2'-OH of the remaining nucleotides is replaced by methoxy group.
aatgagcctcgataactctgt

SEQ ID NO: 528 - RNA, 21 nt, synthetic construct
  source 1..21: mol_type = other RNA
  misc_feature 1..3: note = modified _base - linked via monothioate phosphorodiester bond
  misc_feature 19..21: note = modified _base - linked via monothioate phosphorodiester bond
  misc_feature 1..21: note = 2'-OH of the nucleotides at positions 9,10,11 from the 5' end is replaced by fluorine, 2'-OH of the remaining nucleotides is replaced by methoxy group.
acagagttatcgaggctcatt

SEQ ID NO: 529 - RNA, 21 nt, synthetic construct
  source 1..21: mol_type = other RNA
  misc_feature 20..21: note = T is dT
  misc_feature 1..3: note = modified _base - linked via monothioate phosphorodiester bond
  misc_feature 19..21: note = modified _base - linked via monothioate phosphorodiester bond
  misc_feature 1..19: note = 2'-OH of the nucleotides at positions 2,6,8,14,16 from the 5' end is replaced by fluorine, 2'-OH of the remaining nucleotides is replaced by methoxy group.
tataacaataaggagctgctt

SEQ ID NO: 530 - RNA, 19 nt, synthetic construct
  source 1..19: mol_type = other RNA
  misc_difference 19: note = linked to L96 via monothioate phosphorodiester bond
  misc_feature 1..3: note = modified _base - linked via monothioate phosphorodiester bond
  misc_feature 18..19: note = modified _base - linked via monothioate phosphorodiester bond
  misc_feature 1..19: note = 2'-OH of the nucleotides at positions 7,8,9 from the 5' end is replaced by fluorine, 2'-OH of the remaining nucleotides is replaced by methoxy group.
gcagctccttattgttata

SEQ ID NO: 531 - RNA, 21 nt, synthetic construct
  source 1..21: mol_type = other RNA
  misc_feature 20..21: note = T is dT
  misc_feature 1..3: note = modified _base - linked via monothioate phosphorodiester bond
  misc_feature 1: note = modified with 5'-(E)-vinylphosphonate group
  misc_feature 19..21: note = modified _base - linked via monothioate phosphorodiester bond
  misc_feature 1..19: note = 2'-OH of the nucleotides at positions 2,6,8,14,16 from the 5' end is replaced by fluorine, 2'-OH of the remaining nucleotides is replaced by methoxy group.
tataacaataaggagctgctt

SEQ ID NO: 532 - RNA, 19 nt, synthetic construct
  source 1..19: mol_type = other RNA
  misc_difference 19: note = linked to L96 via monothioate phosphorodiester bond
  misc_feature 1..3: note = modified _base - linked via monothioate phosphorodiester bond
  misc_feature 18..19: note = modified _base - linked via monothioate phosphorodiester bond
  misc_feature 1..19: note = 2'-OH of the nucleotides at positions 7,8,9 from the 5' end is replaced by fluorine, 2'-OH of the remaining nucleotides is replaced by methoxy group.
gcagctccttattgttata

SEQ ID NO: 533 - RNA, 21 nt, synthetic construct
  source 1..21: mol_type = other RNA
  misc_feature 1..3: note = modified _base - linked via monothioate phosphorodiester bond
  misc_feature 19..21: note = modified _base - linked via monothioate phosphorodiester bond
  misc_feature 1..21: note = 2'-OH of the nucleotides at positions 2,4,6,12,14,16 from the 5' end is replaced by fluorine, 2'-OH of the remaining nucleotides is replaced by methoxy group.
aagggcgaatctcagcatctg

SEQ ID NO: 534 - RNA, 21 nt, synthetic construct
  source 1..21: mol_type = other RNA
  misc_feature 21: note = linked to L96 via monothioate phosphorodiester bond
  misc_feature 1..3: note = modified _base - linked via monothioate phosphorodiester bond
  misc_feature 19..21: note = modified _base - linked via monothioate phosphorodiester bond
  misc_feature 1..21: note = 2'-OH of the nucleotides at positions 9,10,11 from the 5' end is replaced by fluorine, 2'-OH of the remaining nucleotides is replaced by methoxy group.
cagatgctgagattcgccctt

SEQ ID NO: 535 - RNA, 21 nt, synthetic construct
  source 1..21: mol_type = other RNA
  misc_feature 1..3: note = modified _base - linked via monothioate phosphorodiester bond
  misc_feature 1: note = modified with 5'-(E)-vinylphosphonate group
  misc_feature 19..21: note = modified _base - linked via monothioate phosphorodiester bond
  misc_feature 1..21: note = 2'-OH of the nucleotides at positions 2,4,6,12,14,16 from the 5' end is replaced by fluorine, 2'-OH of the remaining nucleotides is replaced by methoxy group.
aagggcgaatctcagcatctg

SEQ ID NO: 536 - RNA, 21 nt, synthetic construct
  source 1..21: mol_type = other RNA
  misc_feature 21: note = linked to L96 via monothioate phosphorodiester bond
  misc_feature 1..3: note = modified _base - linked via monothioate phosphorodiester bond
  misc_feature 19..21: note = modified _base - linked via monothioate phosphorodiester bond
  misc_feature 1..21: note = 2'-OH of the nucleotides at positions 9,10,11 from the 5' end is replaced by fluorine, 2'-OH of the remaining nucleotides is replaced by methoxy group.
cagatgctgagattcgccctt

SEQ ID NO: 537 - RNA, 21 nt, synthetic construct
  source 1..21: mol_type = other RNA
  misc_feature 1..3: note = modified _base - linked via monothioate phosphorodiester bond
  misc_feature 19..21: note = modified _base - linked via monothioate phosphorodiester bond
  misc_feature 1..21: note = 2'-OH of the nucleotides at positions 2,4,6,12,14,16 from the 5' end is replaced by fluorine, 2'-OH of the remaining nucleotides is replaced by methoxy group.
aatgagcctcgataactctgt

SEQ ID NO: 538 - RNA, 21 nt, synthetic construct
  source 1..21: mol_type = other RNA
  misc_feature 21: note = linked to L96 via monothioate phosphorodiester bond
  misc_feature 1..3: note = modified _base - linked via monothioate phosphorodiester bond
  misc_feature 19..21: note = modified _base - linked via monothioate phosphorodiester bond
  misc_feature 1..21: note = 2'-OH of the nucleotides at positions 9,10,11 from the 5' end is replaced by fluorine, 2'-OH of the remaining nucleotides is replaced by methoxy group.
acagagttatcgaggctcatt

SEQ ID NO: 539 - RNA, 21 nt, synthetic construct
  source 1..21: mol_type = other RNA
  misc_feature 1..3: note = modified _base - linked via monothioate phosphorodiester bond
  misc_feature 1: note = modified with 5'-(E)-vinylphosphonate group
  misc_feature 19..21: note = modified _base - linked via monothioate phosphorodiester bond
  misc_feature 1..21: note = 2'-OH of the nucleotides at positions 2,4,6,12,14,16 from the 5' end is replaced by fluorine, 2'-OH of the remaining nucleotides is replaced by methoxy group.
aatgagcctcgataactctgt

SEQ ID NO: 540 - RNA, 21 nt, synthetic construct
  source 1..21: mol_type = other RNA
  misc_feature 21: note = linked to L96 via monothioate phosphorodiester bond
  misc_feature 1..3: note = modified _base - linked via monothioate phosphorodiester bond
  misc_feature 19..21: note = modified _base - linked via monothioate phosphorodiester bond
  misc_feature 1..21: note = 2'-OH of the nucleotides at positions 9,10,11 from the 5' end is replaced by fluorine, 2'-OH of the remaining nucleotides is replaced by methoxy group.
acagagttatcgaggctcatt

SEQ ID NO: 541 - RNA, 19 nt, synthetic construct
  source 1..19: mol_type = other RNA
gtggcagctccttattgtt

SEQ ID NO: 542 - RNA, 19 nt, synthetic construct
  source 1..19: mol_type = other RNA
gcagctccttattgttata

SEQ ID NO: 543 - RNA, 19 nt, synthetic construct
  source 1..19: mol_type = other RNA
gcttgatcaagaactactg

SEQ ID NO: 544 - RNA, 21 nt, synthetic construct
  source 1..21: mol_type = other RNA
  misc_feature 20..21: note = T is dT
aacaataaggagctgccactt

SEQ ID NO: 545 - RNA, 21 nt, synthetic construct
  source 1..21: mol_type = other RNA
  misc_feature 20..21: note = T is dT
tataacaataaggagctgctt

SEQ ID NO: 546 - RNA, 21 nt, synthetic construct
  source 1..21: mol_type = other RNA
  misc_feature 20..21: note = T is dT
cagtagttcttgatcaagctt

SEQ ID NO: 547 - RNA, 21 nt, synthetic construct
  source 1..21: mol_type = other RNA
  misc_feature 20..21: note = T is dT
  misc_feature 1..3: note = modified _base - linked via monothioate phosphorodiester bond
  misc_feature 19..21: note = modified _base - linked via monothioate phosphorodiester bond
  misc_feature 1..19: note = 2'-OH of the nucleotides at positions 7,9,10,11,14,16 from the 5' end is replaced by fluorine, 2'-OH of the remaining nucleotides is replaced by methoxy group.
gcagctccttattgttatatt

SEQ ID NO: 548 - RNA, 21 nt, synthetic construct
  source 1..21: mol_type = other RNA
  misc_feature 20..21: note = T is dT
  misc_feature 1..3: note = modified _base - linked via monothioate phosphorodiester bond
  misc_feature 1: note = modified with 5'-(E)-vinylphosphonate group
  misc_feature 19..21: note = modified _base - linked via monothioate phosphorodiester bond
  misc_feature 1..19: note = 2'-OH of the nucleotides at positions 2,4,6,8,14,16 from the 5' end is replaced by fluorine, 2'-OH of the remaining nucleotides is replaced by methoxy group.
tataacaataaggagctgctt

SEQ ID NO: 549 - RNA, 21 nt, synthetic construct
  source 1..21: mol_type = other RNA
  misc_feature 1..3: note = modified _base - linked via monothioate phosphorodiester bond
  misc_feature 19..21: note = modified _base - linked via monothioate phosphorodiester bond
  misc_feature 1..21: note = 2'-OH of the nucleotides at positions 7,9,10,11,14,16 from the 5' end is replaced by fluorine, 2'-OH of the remaining nucleotides is replaced by methoxy group.
tggcagctccttattgttata

SEQ ID NO: 550 - RNA, 23 nt, synthetic construct
  source 1..23: mol_type = other RNA
  misc_feature 1..3: note = modified _base - linked via monothioate phosphorodiester bond
  misc_feature 21..23: note = modified _base - linked via monothioate phosphorodiester bond
  misc_feature 1..23: note = 2'-OH of the nucleotides at positions 2,6,14,16 from the 5' end is replaced by fluorine, 2'-OH of the remaining nucleotides is replaced by methoxy group.
tataacaataaggagctgccaca

SEQ ID NO: 551 - RNA, 21 nt, synthetic construct
  source 1..21: mol_type = other RNA
  misc_feature 1: note = linked to NAG25 via monothioate phosphorodiester bond
  misc_feature 1..2: note = modified _base - linked via monothioate phosphorodiester bond
  misc_feature 20..21: note = modified with monothioate phosphorodiester bond
  misc_feature 21: note = inverted nucleotide
  misc_feature 1..20: note = 2'-OH of the nucleotides at positions 9,10,11 from the 5' end is replaced by fluorine, 2'-OH of the remaining nucleotides is replaced by methoxy group.
cagccccttattgttatacga

SEQ ID NO: 552 - RNA, 21 nt, synthetic construct
  source 1..21: mol_type = other RNA
  misc_feature 1..3: note = modified _base - linked via monothioate phosphorodiester bond
  misc_feature 19..21: note = modified _base - linked via monothioate phosphorodiester bond
  misc_feature 1..21: note = 2'-OH of the nucleotides at positions 2,4,6,12,14,16 from the 5' end is replaced by fluorine, 2'-OH of the remaining nucleotides is replaced by methoxy group.
tcgtataacaataaggggctg

SEQ ID NO: 553 - RNA, 19 nt, synthetic construct
  source 1..19: mol_type = other RNA
  misc_feature 1: note = linked to [ST23*]3/C6XLT via a phosphorothioate diester bond
  misc_feature 17..19: note = modified _base - linked via monothioate phosphorodiester bond
  misc_feature 1..19: note = 2'-OH of the nucleotides at positions 7,8,9 from the 5' end is replaced by fluorine, 2'-OH of the remaining nucleotides is replaced by methoxy group.
cggtaatggacagagttat

SEQ ID NO: 554 - RNA, 19 nt, synthetic construct
  source 1..19: mol_type = other RNA
  misc_feature 1..3: note = modified _base - linked via monothioate phosphorodiester bond
  misc_feature 17..19: note = modified _base - linked via monothioate phosphorodiester bond
  misc_feature 1..19: note = 2'-OH of the nucleotides at positions 2,4,6,8,14,16 from the 5' end is replaced by fluorine, 2'-OH of the remaining nucleotides is replaced by methoxy group.
ataactctgtccattaccg

SEQ ID NO: 555 - RNA, 21 nt, synthetic construct
  source 1..21: mol_type = other RNA
cagccccttattgttatacga

SEQ ID NO: 556 - RNA, 21 nt, synthetic construct
  source 1..21: mol_type = other RNA
tcgtataacaataaggggctg

SEQ ID NO: 557 - RNA, 21 nt, synthetic construct
  source 1..21: mol_type = other RNA
  misc_feature 20..21: note = T is dT
  misc_feature 1..3: note = modified _base - linked via monothioate phosphorodiester bond
  misc_feature 1: note = modified with 5'-(E)-vinylphosphonate group
  misc_feature 19..21: note = modified _base - linked via monothioate phosphorodiester bond
  misc_feature 21: note = linked to biotin
  misc_feature 1..19: note = 2'-OH of the nucleotides at positions 2,6,8,14,16 from the 5' end is replaced by fluorine, 2'-OH of the remaining nucleotides is replaced by methoxy group.
tataacaataaggagctgctt

SEQ ID NO: 558 - RNA, 21 nt, synthetic construct
  source 1..21: mol_type = other RNA
  misc_feature 20..21: note = T is dT
  misc_feature 1..3: note = modified _base - linked via monothioate phosphorodiester bond
  misc_feature 1: note = modified with 5'-(E)-vinylphosphonate group
  misc_feature 19..21: note = modified _base - linked via monothioate phosphorodiester bond
  misc_feature 21: note = linked to biotin
  misc_feature 1..19: note = 2'-OH of the nucleotides at positions 2,4,6,8,14,16 from the 5' end is replaced by fluorine, 2'-OH of the remaining nucleotides is replaced by methoxy group.
tataacaataaggagctgctt

SEQ ID NO: 559 - RNA, 23 nt, synthetic construct
  source 1..23: mol_type = other RNA
  misc_feature 1..3: note = modified _base - linked via monothioate phosphorodiester bond
  misc_feature 21..23: note = modified _base - linked via monothioate phosphorodiester bond
  misc_feature 23: note = linked to biotin
  misc_feature 1..23: note = 2'-OH of the nucleotides at positions 2,6,14,16 from the 5' end is replaced by fluorine, 2'-OH of the remaining nucleotides is replaced by methoxy group.
tataacaataaggagctgccaca

SEQ ID NO: 560 - RNA, 21 nt, synthetic construct
  source 1..21: mol_type = other RNA
  misc_feature 20..21: note = T is dT
  misc_feature 1..3: note = modified _base - linked via monothioate phosphorodiester bond
  misc_feature 19..21: note = modified _base - linked via monothioate phosphorodiester bond
  misc_feature 21: note = linked to biotin
  misc_feature 1..19: note = 2'-OH of the nucleotides at positions 2,6,8,14,16 from the 5' end is replaced by fluorine, 2'-OH of the remaining nucleotides is replaced by methoxy group.
tataacaataaggagctgctt